European Patent Specification EP 3 510 157 B1, published May 31, 2023. Title: PD-1 HOMING ENDONUCLEASE VARIANTS, COMPOSITIONS, AND METHODS OF USE. Applicant: bluebird bio, Inc. Mann, Jasdeep Gay, Joel Jarjour, Jordan Zhang, Joy. The sequence listing filed with the application follows.

SEQUENCE LISTING (123 sequences)

SEQ ID NO: 1 - protein, 303 aa, Ophiostoma novo-ulmi subsp. americana (mitochondrion)
MAYMSRRESINPWILTGFADAEGSFLLRIRNNNKSSVGYSTELGFQITLHNKDKSILENIQSTWKVGVIANSGDNAVSLKVTRFEDLKVIIDHFEKYPLITQKLGDYMLFKQAFCVMENKEHLKINGIKELVRIKAKLNWGLTDELKKAFPEIISKERSLINKNIPNFKWLAGFTSGEGCFFVNLIKSKSKLGVQVQLVFSITQHIKDKNLMNSLITYLGCGYIKEKNKSEFSWLDFVVTKFSDINDKIIPVFQENTLIGVKLEDFEDWCKVAKLIEEKKHLTESGLDEIKKIKLNMNKGRVF

SEQ ID NO: 2 - protein, 303 aa, Ophiostoma novo-ulmi subsp. americana (mitochondrion)
MAYMSRRESINPWILTGFADAEGSFLLRIRNNNKSSVGYSTELGFQITLHNKDKSILENIQSTWKVGVIANSGDNAVSLKVTRFEDLKVIIDHFEKYPLITQKLGDYKLFKQAFSVMENKEHLKENGIKELVRIKAKLNWGLTDELKKAFPENISKERSLINKNIPNFKWLAGFTSGEGCFFVNLIKSKSKLGVQVQLVFSITQHIKDKNLMNSLITYLGCGYIKEKNKSEFSWLDFVVTKFSDINDKIIPVFQENTLIGVKLEDFEDWCKVAKLIEEKKHLTESGLDEIKKIKLNMNKGRVF

SEQ ID NO: 3 - protein, 303 aa, Ophiostoma novo-ulmi subsp. americana (mitochondrion)
  MOD_RES (1)..(3): Any amino acid or absent
XXXMSRRESINPWILTGFADAEGSFLLRIRNNNKSSVGYSTELGFQITLHNKDKSILENIQSTWKVGVIANSGDNAVSLKVTRFEDLKVIIDHFEKYPLITQKLGDYKLFKQAFSVMENKEHLKENGIKELVRIKAKLNWGLTDELKKAFPENISKERSLINKNIPNFKWLAGFTSGEGCFFVNLIKSKSKLGVQVQLVFSITQHIKDKNLMNSLITYLGCGYIKEKNKSEFSWLDFVVTKFSDINDKIIPVFQENTLIGVKLEDFEDWCKVAKLIEEKKHLTESGLDEIKKIKLNMNKGRVF

SEQ ID NO: 4 - protein, 303 aa, Ophiostoma novo-ulmi subsp. americana (mitochondrion)
  MOD_RES (1)..(4): Any amino acid or absent
  MOD_RES (302)..(303): Any amino acid or absent
XXXXSRRESINPWILTGFADAEGSFLLRIRNNNKSSVGYSTELGFQITLHNKDKSILENIQSTWKVGVIANSGDNAVSLKVTRFEDLKVIIDHFEKYPLITQKLGDYKLFKQAFSVMENKEHLKENGIKELVRIKAKLNWGLTDELKKAFPENISKERSLINKNIPNFKWLAGFTSGEGCFFVNLIKSKSKLGVQVQLVFSITQHIKDKNLMNSLITYLGCGYIKEKNKSEFSWLDFVVTKFSDINDKIIPVFQENTLIGVKLEDFEDWCKVAKLIEEKKHLTESGLDEIKKIKLNMNKGRXX

SEQ ID NO: 5 - protein, 303 aa, Ophiostoma novo-ulmi subsp. americana (mitochondrion)
  MOD_RES (1)..(8): Any amino acid or absent
  MOD_RES (302)..(303): Any amino acid or absent
XXXXXXXXSINPWILTGFADAEGSFLLRIRNNNKSSVGYSTELGFQITLHNKDKSILENIQSTWKVGVIANSGDNAVSLKVTRFEDLKVIIDHFEKYPLITQKLGDYKLFKQAFSVMENKEHLKENGIKELVRIKAKLNWGLTDELKKAFPENISKERSLINKNIPNFKWLAGFTSGEGCFFVNLIKSKSKLGVQVQLVFSITQHIKDKNLMNSLITYLGCGYIKEKNKSEFSWLDFVVTKFSDINDKIIPVFQENTLIGVKLEDFEDWCKVAKLIEEKKHLTESGLDEIKKIKLNMNKGRXX

SEQ ID NO: 6 - protein, 303 aa, Artificial Sequence
  Synthesized I-OnuI variant PD-1.ITSM.ex5_RD1_CV3-08
  MOD_RES (1)..(4): Any amino acid or absent
  MOD_RES (302)..(303): Any amino acid or absent
XXXXSRRESINPWILTGFADAEGSFQLEIRNVNPNIPRYKTRLRFEIDLHNKDKSILENIQSTWKVGKIYNQGDSYVKLRVTRFEDLKVIIDHFEKYPLITQKLGDYKLFKQAFSVMENKEHLKENGIKELVRIKAKMNWGLNDELKKAFPENISKERPLINKNIPNLKWLAGFTSGEGHFGVILAKRRPASPVQVRLRFAIGQHIRDKNLMNSLITYLGCGRIREKNISEKSWLEFEVTKFSDINDKIIPVFQENTLIGVKLEDFEDWCKVAKLIEEKKHLTESGLDEIKKIKLNMNKGRXX

SEQ ID NO: 7 - protein, 303 aa, Artificial Sequence
  Synthesized I-OnuI variant PD-1.ITSM.ex5_RD2_73
  MOD_RES (1)..(4): Any amino acid or absent
  MOD_RES (302)..(303): Any amino acid or absent
XXXXSRRESINPWILTGFADAEGSFQLEIRNVNPNIPRYRTRLRFEIDLHNKDKSILEDIQSTWKVGKIYNRGDSYVKLRVTRFEDLKVIIDHFEKYPLITQKLGDYKLFKQAFSVMENKEHLKENGIKELVRIKAKMNWGLNDELKKAFPENISKERPLINKNIPNLKWLAGFTSGEGHFGVILAKRRPASPVQVRLRFAIGQHIRDKNLMNSLITYLGCGRTREKNISEKSWLEFEVTKFSDINDKIIPVFQENTLIGVKLEDFEDWCKVAKLIEEKKHLTESGLDEIKKIKLNMNKGRXX

SEQ ID NO: 8 - protein, 303 aa, Artificial Sequence
  Synthesized I-OnuI variant PD-1.ITSM.ex5_RD3_03
  MOD_RES (1)..(4): Any amino acid or absent
  MOD_RES (302)..(303): Any amino acid or absent
XXXXSRRESINPWILTGFADAEGSFQLEIRNVNPNIPRYRTRLRFEIDLHNKDKSILEDIQSTWKVGKIYNQGDSYVKLRVTRFEDLKVIIDHFEKYPLITQKLGDYKLFKQAFSVMENKEHLKENGIKELVRIKAKMNWGLNDELKKAFPENISKERPLINKNIPNLKWLAGFTSGDGHFGVILAKRRPASPVQVRLRFAIGQHIRDKNLMNSLITYLGCGRTREKNISEKSWLEFEVTKFSDINDKIIPVFQENTLIGVKLEDFEDWCKVAKLIEEKKHLTESGLDEIKKIKLNMNKGRXX

SEQ ID NO: 9 - protein, 303 aa, Artificial Sequence
  Synthesized I-OnuI variant PD-1.ITSM.ex5_RD4_CV23
  MOD_RES (1)..(4): Any amino acid or absent
  MOD_RES (302)..(303): Any amino acid or absent
XXXXSRRESINPWILTGFADAEGSFQLEIRNVNPNIPRYRTRLRFEIDLHNKDKSILEDIQSTWKVGKIYNQGDSYVKLRVTRFEDLKVIIDHFEKYPLITQKLGDYKLFKQAFSVMENKEHLKENGIKELVRIKAKMNWGLNDELKKAFPENISKERPLINKNIPNLKWLAGFTSGDGHFGVILAKRRPASPVQVRLRFAIGQHIRDKNLMNSLITYLGCGRIREKNKSEKSWLEFEVTKFSDINDKIIPVFQENTLIGVKLEDFEDWCKVAKLIEEKKHLTESGLDEIKKIKLNMNKGRXX

SEQ ID NO: 10 - protein, 303 aa, Artificial Sequence
  Synthesized I-OnuI variant PD-1.ITSM.ex5_RD5_CV23MK
  MOD_RES (1)..(4): Any amino acid or absent
  MOD_RES (302)..(303): Any amino acid or absent
XXXXSRRESINPWILTGFADAEGSFQLEIRNVNPNIPRYRTRLRFEIDLHNKDKSILEDIQSTWKVGKIYNQGDSYVKLRVTRFEDLKVIIDHFEKYPLITQKLGDYKLFKQAFSVMENKEHLKENGIKELVRIKAKMNWGLNDELKKAFPENISKERPLINKNIPNLKWLAGFTSGDGHFGVILAKRRPASPVQVRLRFMIGQHIKDKNLMNSLITYLGCGRIREKNKSEKSWLEFEVTKFSDINDKIIPVFQENTLIGVKLEDFEDWCKVAKLIEEKKHLTESGLDEIKKIKLNMNKGRXX

SEQ ID NO: 11 - protein, 303 aa, Artificial Sequence
  Synthesized I-OnuI variant PD-1.ile3.exon1_RD1_B1
  MOD_RES (1)..(4): Any amino acid or absent
  MOD_RES (302)..(303): Any amino acid or absent
XXXXSRRESINPWILTGFADAEGSFGLSILNRNRGTARYHTRLSFAIVLHNKDKSILENIQSTWKVGIITNDGDRYVRLRVTRFEDLKVIIDHFEKYPLVTQKLGDYKLFKQAFSVMENKEHLKENGIKELVRIKAKMNWGLNDELKKAFPENISKERPLINKNIPNFKWLAGFTSGDGSFFVRLRKSNVNARVRVQLVFEISQHIRDKNLMNSLITYLGCGHIYEGNKSERSWLQFRVEKFSDINDKIIPVFQENTLIGVKLEDFEDWCKVAKLIEEKKHLTESGLDEIKKIKLNMNKGRXX

SEQ ID NO: 12 - protein, 303 aa, Artificial Sequence
  Synthesized I-OnuI variant PD-1.ile3.exon1_RD2_B1H8
  MOD_RES (1)..(4): Any amino acid or absent
  MOD_RES (302)..(303): Any amino acid or absent
XXXXSRRESINPWILTGFADAEGSFGLSILNRNRGTARYHTRLSFTIVLHNKDKSILENIQSTWKVGIITNDGDRYVRLCVTRFEDLKVIIDHFEKYPLVTQKLGDYKLFKQAFSVMENKEHLKENGIKELARIKAKMNWGLNDELKKAFPENIGKERPLINKNIPNFKWLAGFTSGDGSFFVRLRKSNVNARVRVQLVFEISQHIRDKNLMNSLITYLGCGHIYEGNKSERSWLQFRVEKFSDINDKIIPVFQENTLIGVKLEDFEDWCKVAKLIEEKKHLTESGLDEIKKIKLNMNKGRXX

SEQ ID NO: 13 - protein, 303 aa, Artificial Sequence
  Synthesized I-OnuI variant PD-1.IgV.exon2_RD1_G5
  MOD_RES (1)..(4): Any amino acid or absent
  MOD_RES (302)..(303): Any amino acid or absent
XXXXSRRESINPWILTGFADAEGSFQLYISNVNNNRSRYRARLRFAIELHNKDKSILENIQSTWKVGVINNIGDTSVRLSVGRFEDLKVIIDHFEKYPLITQKLGDYKLFKQAFSVMENKEHLKENGIKELVRIKAKMNWGLNDELKKAFPENISKERPLINKNIPNLKWLAGFTSGDGNFYVHLKKSGRTTRVYVQLRFSIAQHIRDKNLMNSLITYLGCGYINEWNASERSALEFRVTKFSDINDKIIPVFQENTLIGVKLEDFEDWCKVAKLIEEKKHLTESGLDEIKKIKLNMNKGRXX

SEQ ID NO: 14 - protein, 303 aa, Artificial Sequence
  Synthesized I-OnuI variant PD-1.IgV.exon2_RD1_PS3
  MOD_RES (1)..(4): Any amino acid or absent
  MOD_RES (302)..(303): Any amino acid or absent
XXXXSRRESINPWILTGFADAEGCFLLHIRNLNRTSTKYRTRLSFEIELHNKDKSILENIQSTWKVGIINNIGNRRVRLSVRRFEDLKVIIDHFEKYPLITQKLGDYKLFKQAFSLMENKEHLKENGIKELVRIKAKMNWGLNDELKKAFPENISKERPLINKNIPNLKWLAGFTSGDGNFYVHLKKSGRTTRVYVQLRFSISQHIRDKNLMNSLITYLGCGYITESNPSERSDLEFRVTKFSDINDKIIPVFQENTLIGVKLEDFEDWCKVAKLIEEKKHLTESGLDEIKKIKLNMNKGRXX

SEQ ID NO: 15 - protein, 870 aa, Artificial Sequence
  Synthesized megaTAL PD-1.ITSM.ex5_RD1_CV3-08
MGSAPPKKKRKVVDLRTLGYSQQQQEKIKPKVRSTVAQHHEALVGHGFTHAHIVALSQHPAALGTVAVTYQHIITALPEATHEDIVGVGKQWSGARALEALLTDAGELRGPPLQLDTGQLVKIAKRGGVTAMEAVHASRNALTGAPLNLTPDQVVAIASNGGGKQALETVQRLLPVLCQDHGLTPDQVVAIASHDGGKQALETVQRLLPVLCQDHGLTPDQVVAIASNGGKQALETVQRLLPVLCQDHGLTPDQVVAIASNNGGKQALETVQRLLPVLCQDHGLTPDQVVAIASHDGGKQALETVQRLLPVLCQDHGLTPDQVVAIASNGGGKQALETVQRLLPVLCQDHGLTPDQVVAIASNIGGKQALETVQRLLPVLCQDHGLTPDQVVAIASNNGGKQALETVQRLLPVLCQDHGLTPDQVVAIASNNGGKQALETVQRLLPVLCQDHGLTPDQVVAIASNIGGKQALETVQRLLPVLCQDHGLTPDQVVAIASNIGGKQALESIVAQLSRPDPALAALTNDHLVALACLGGRPAMDAVKKGLPHAPELIRRVNRRIGERTSHRVAISRSRRESINPWILTGFADAEGSFQLEIRNVNPNIPRYKTRLRFEIDLHNKDKSILENIQSTWKVGKIYNQGDSYVKLRVTRFEDLKVIIDHFEKYPLITQKLGDYKLFKQAFSVMENKEHLKENGIKELVRIKAKMNWGLNDELKKAFPENISKERPLINKNIPNLKWLAGFTSGEGHFGVILAKRRPASPVQVRLRFAIGQHIRDKNLMNSLITYLGCGRIREKNISEKSWLEFEVTKFSDINDKIIPVFQENTLIGVKLEDFEDWCKVAKLIEEKKHLTESGLDEIKKIKLNMNKGR

SEQ ID NO: 16 - protein, 870 aa, Artificial Sequence
  Synthesized megaTAL PD-1.ITSM.ex5_RD2_73
MGSAPPKKKRKVVDLRTLGYSQQQQEKIKPKVRSTVAQHHEALVGHGFTHAHIVALSQHPAALGTVAVTYQHIITALPEATHEDIVGVGKQWSGARALEALLTDAGELRGPPLQLDTGQLVKIAKRGGVTAMEAVHASRNALTGAPLNLTPDQVVAIASNGGGKQALETVQRLLPVLCQDHGLTPDQVVAIASHDGGKQALETVQRLLPVLCQDHGLTPDQVVAIASNGGKQALETVQRLLPVLCQDHGLTPDQVVAIASNNGGKQALETVQRLLPVLCQDHGLTPDQVVAIASHDGGKQALETVQRLLPVLCQDHGLTPDQVVAIASNGGGKQALETVQRLLPVLCQDHGLTPDQVVAIASNIGGKQALETVQRLLPVLCQDHGLTPDQVVAIASNNGGKQALETVQRLLPVLCQDHGLTPDQVVAIASNNGGKQALETVQRLLPVLCQDHGLTPDQVVAIASNIGGKQALETVQRLLPVLCQDHGLTPDQVVAIASNIGGKQALESIVAQLSRPDPALAALTNDHLVALACLGGRPAMDAVKKGLPHAPELIRRVNRRIGERTSHRVAISRSRRESINPWILTGFADAEGSFQLEIRNVNPNIPRYRTRLRFEIDLHNKDKSILEDIQSTWKVGKIYNRGDSYVKLRVTRFEDLKVIIDHFEKYPLITQKLGDYKLFKQAFSVMENKEHLKENGIKELVRIKAKMNWGLNDELKKAFPENISKERPLINKNIPNLKWLAGFTSGEGHFGVILAKRRPASPVQVRLRFAIGQHIRDKNLMNSLITYLGCGRTREKNISEKSWLEFEVTKFSDINDKIIPVFQENTLIGVKLEDFEDWCKVAKLIEEKKHLTESGLDEIKKIKLNMNKGR

SEQ ID NO: 17 - protein, 870 aa, Artificial Sequence
  Synthesized megaTAL PD-1.ITSM.ex5_RD3_03
MGSAPPKKKRKVVDLRTLGYSQQQQEKIKPKVRSTVAQHHEALVGHGFTHAHIVALSQHPAALGTVAVTYQHIITALPEATHEDIVGVGKQWSGARALEALLTDAGELRGPPLQLDTGQLVKIAKRGGVTAMEAVHASRNALTGAPLNLTPDQVVAIASNGGGKQALETVQRLLPVLCQDHGLTPDQVVAIASHDGGKQALETVQRLLPVLCQDHGLTPDQVVAIASNGGKQALETVQRLLPVLCQDHGLTPDQVVAIASNNGGKQALETVQRLLPVLCQDHGLTPDQVVAIASHDGGKQALETVQRLLPVLCQDHGLTPDQVVAIASNGGGKQALETVQRLLPVLCQDHGLTPDQVVAIASNIGGKQALETVQRLLPVLCQDHGLTPDQVVAIASNNGGKQALETVQRLLPVLCQDHGLTPDQVVAIASNNGGKQALETVQRLLPVLCQDHGLTPDQVVAIASNIGGKQALETVQRLLPVLCQDHGLTPDQVVAIASNIGGKQALESIVAQLSRPDPALAALTNDHLVALACLGGRPAMDAVKKGLPHAPELIRRVNRRIGERTSHRVAISRSRRESINPWILTGFADAEGSFQLEIRNVNPNIPRYRTRLRFEIDLHNKDKSILEDIQSTWKVGKIYNQGDSYVKLRVTRFEDLKVIIDHFEKYPLITQKLGDYKLFKQAFSVMENKEHLKENGIKELVRIKAKMNWGLNDELKKAFPENISKERPLINKNIPNLKWLAGFTSGDGHFGVILAKRRPASPVQVRLRFAIGQHIRDKNLMNSLITYLGCGRTREKNISEKSWLEFEVTKFSDINDKIIPVFQENTLIGVKLEDFEDWCKVAKLIEEKKHLTESGLDEIKKIKLNMNKGR

SEQ ID NO: 18 - protein, 870 aa, Artificial Sequence
  Synthesized megaTAL PD-1.ITSM.ex5_RD4_CV23
MGSAPPKKKRKVVDLRTLGYSQQQQEKIKPKVRSTVAQHHEALVGHGFTHAHIVALSQHPAALGTVAVTYQHIITALPEATHEDIVGVGKQWSGARALEALLTDAGELRGPPLQLDTGQLVKIAKRGGVTAMEAVHASRNALTGAPLNLTPDQVVAIASNGGGKQALETVQRLLPVLCQDHGLTPDQVVAIASHDGGKQALETVQRLLPVLCQDHGLTPDQVVAIASNGGKQALETVQRLLPVLCQDHGLTPDQVVAIASNNGGKQALETVQRLLPVLCQDHGLTPDQVVAIASHDGGKQALETVQRLLPVLCQDHGLTPDQVVAIASNGGGKQALETVQRLLPVLCQDHGLTPDQVVAIASNIGGKQALETVQRLLPVLCQDHGLTPDQVVAIASNNGGKQALETVQRLLPVLCQDHGLTPDQVVAIASNNGGKQALETVQRLLPVLCQDHGLTPDQVVAIASNIGGKQALETVQRLLPVLCQDHGLTPDQVVAIASNIGGKQALESIVAQLSRPDPALAALTNDHLVALACLGGRPAMDAVKKGLPHAPELIRRVNRRIGERTSHRVAISRSRRESINPWILTGFADAEGSFQLEIRNVNPNIPRYRTRLRFEIDLHNKDKSILEDIQSTWKVGKIYNQGDSYVKLRVTRFEDLKVIIDHFEKYPLITQKLGDYKLFKQAFSVMENKEHLKENGIKELVRIKAKMNWGLNDELKKAFPENISKERPLINKNIPNLKWLAGFTSGDGHFGVILAKRRPASPVQVRLRFAIGQHIRDKNLMNSLITYLGCGRIREKNKSEKSWLEFEVTKFSDINDKIIPVFQENTLIGVKLEDFEDWCKVAKLIEEKKHLTESGLDEIKKIKLNMNKGR

SEQ ID NO: 19 - protein, 870 aa, Artificial Sequence
  Synthesized megaTAL PD-1.ITSM.ex5_RD5_CV23MK
MGSAPPKKKRKVVDLRTLGYSQQQQEKIKPKVRSTVAQHHEALVGHGFTHAHIVALSQHPAALGTVAVTYQHIITALPEATHEDIVGVGKQWSGARALEALLTDAGELRGPPLQLDTGQLVKIAKRGGVTAMEAVHASRNALTGAPLNLTPDQVVAIASNGGGKQALETVQRLLPVLCQDHGLTPDQVVAIASHDGGKQALETVQRLLPVLCQDHGLTPDQVVAIASNGGKQALETVQRLLPVLCQDHGLTPDQVVAIASNNGGKQALETVQRLLPVLCQDHGLTPDQVVAIASHDGGKQALETVQRLLPVLCQDHGLTPDQVVAIASNGGGKQALETVQRLLPVLCQDHGLTPDQVVAIASNIGGKQALETVQRLLPVLCQDHGLTPDQVVAIASNNGGKQALETVQRLLPVLCQDHGLTPDQVVAIASNNGGKQALETVQRLLPVLCQDHGLTPDQVVAIASNIGGKQALETVQRLLPVLCQDHGLTPDQVVAIASNIGGKQALESIVAQLSRPDPALAALTNDHLVALACLGGRPAMDAVKKGLPHAPELIRRVNRRIGERTSHRVAISRSRRESINPWILTGFADAEGSFQLEIRNVNPNIPRYRTRLRFEIDLHNKDKSILEDIQSTWKVGKIYNQGDSYVKLRVTRFEDLKVIIDHFEKYPLITQKLGDYKLFKQAFSVMENKEHLKENGIKELVRIKAKMNWGLNDELKKAFPENISKERPLINKNIPNLKWLAGFTSGDGHFGVILAKRRPASPVQVRLRFMIGQHIKDKNLMNSLITYLGCGRIREKNKSEKSWLEFEVTKFSDINDKIIPVFQENTLIGVKLEDFEDWCKVAKLIEEKKHLTESGLDEIKKIKLNMNKGR

SEQ ID NO: 20 - protein, 841 aa, Artificial Sequence
  Synthesized megaTAL PD-1.ile3.exon1_RD1 B1
MGSAPPKKKRKVVDLRTLGYSQQQQEKIKPKVRSTVAQHHEALVGHGFTHAHIVALSQHPAALGTVAVTYQHIITALPEATHEDIVGVGKQWSGARALEALLTDAGELRGPPLQLDTGQLVKIAKRGGVTAMEAVHASRNALTGAPLNLTPDQVVAIASNNGGKQALETVQRLLPVLCQDHGLTPDQVVAIASNNGGKQALETVQRLLPVLCQDHGLTPDQVVAIASNGGGKQALETVQRLLPVLCQDHGLTPDQVVAIASNNGGKQALETVQRLLPVLCQDHGLTPDQVVAIASNNGGKQALETVQRLLPVLCQDHGLTPDQVVAIASNNGGKQALETVQRLLPVLCQDHGLTPDQVVAIASNNGGKQALETVQRLLPVLCQDHGLTPDQVVAIASHDGGKQALETVQRLLPVLCQDHGLTPDQVVAIASNGGGKQALETVQRLLPVLCQDHGLTPDQVVAIASNNGGKQALESIVAQLSRPDPALAALTNDHLVALACLGGRPAMDAVKKGLPHAPELIRRVNRRIGERTSHRVAISRVGGSSRRESINPWILTGFADAEGSFGLSILNRNRGTARYHTRLSFAIVLHNKDKSILENIQSTWKVGIITNDGDRYVRLRVTRFEDLKVIIDHFEKYPLVTQKLGDYKLFKQAFSVMENKEHLKENGIKELVRIKAKMNWGLNDELKKAFPENISKERPLINKNIPNFKWLAGFTSGDGSFFVRLRKSNVNARVRVQLVFEISQHIRDKNLMNSLITYLGCGHIYEGNKSERSWLQFRVEKFSDINDKIIPVFQENTLIGVKLEDFEDWCKVAKLIEEKKHLTESGLDEIKKIKLNMNKGR

SEQ ID NO: 21 - protein, 841 aa, Artificial Sequence
  Synthesized megaTAL PD-1.ile3.exon1_RD2_B1H8
MGSAPPKKKRKVVDLRTLGYSQQQQEKIKPKVRSTVAQHHEALVGHGFTHAHIVALSQHPAALGTVAVTYQHIITALPEATHEDIVGVGKQWSGARALEALLTDAGELRGPPLQLDTGQLVKIAKRGGVTAMEAVHASRNALTGAPLNLTPDQVVAIASNNGGKQALETVQRLLPVLCQDHGLTPDQVVAIASNNGGKQALETVQRLLPVLCQDHGLTPDQVVAIASNGGGKQALETVQRLLPVLCQDHGLTPDQVVAIASNNGGKQALETVQRLLPVLCQDHGLTPDQVVAIASNNGGKQALETVQRLLPVLCQDHGLTPDQVVAIASNNGGKQALETVQRLLPVLCQDHGLTPDQVVAIASNNGGKQALETVQRLLPVLCQDHGLTPDQVVAIASHDGGKQALETVQRLLPVLCQDHGLTPDQVVAIASNGGGKQALETVQRLLPVLCQDHGLTPDQVVAIASNNGGKQALESIVAQLSRPDPALAALTNDHLVALACLGGRPAMDAVKKGLPHAPELIRRVNRRIGERTSHRVAISRVGGSSRRESINPWILTGFADAEGSFGLSILNRNRGTARYHTRLSFTIVLHNKDKSILENIQSTWKVGIITNDGDRYVRLCVTRFEDLKVIIDHFEKYPLVTQKLGDYKLFKQAFSVMENKEHLKENGIKELARIKAKMNWGLNDELKKAFPENIGKERPLINKNIPNFKWLAGFTSGDGSFFVRLRKSNVNARVRVQLVFEISQHIRDKNLMNSLITYLGCGHIYEGNKSERSWLQFRVEKFSDINDKIIPVFQENTLIGVKLEDFEDWCKVAKLIEEKKHLTESGLDEIKKIKLNMNKGR

SEQ ID NO: 22 - protein, 909 aa, Artificial Sequence
  Synthesized megaTAL PD-1.IgV.exon2_RD1_G5
MGSAPPKKKRKVVDLRTLGYSQQQQEKIKPKVRSTVAQHHEALVGHGFTHAHIVALSQHPAALGTVAVTYQHIITALPEATHEDIVGVGKQWSGARALEALLTDAGELRGPPLQLDTGQLVKIAKRGGVTAMEAVHASRNALTGAPLNLTPDQVVAIASNNGGKQALETVQRLLPVLCQDHGLTPDQVVAIASNGGGKQALETVQRLLPVLCQDHGLTPDQVVAIASHDGGKQALETVQRLLPVLCQDHGLTPDQVVAIASNIGGKQALETVQRLLPVLCQDHGLTPDQVVAIASHDGGKQALETVQRLLPVLCQDHGLTPDQVVAIASNIGGKQALETVQRLLPVLCQDHGLTPDQVVAIASHDGGKQALETVQRLLPVLCQDHGLTPDQVVAIASNIGGKQALETVQRLLPVLCQDHGLTPDQVVAIASNIGGKQALETVQRLLPVLCQDHGLTPDQVVAIASHDGGKQALETVQRLLPVLCQDHGLTPDQVVAIASNGGGKQALETVQRLLPVLCQDHGLTPDQVVAIASNNGGKQALESIVAQLSRPDPALAALTNDHLVALACLGGRPAMDAVKKGLPHAPELIRRVNRRIGERTSHRVAISRVGGSSRRESINPWILTGFADAEGSFQLYISNVNNNRSRYRARLRFAIELHNKDKSILENIQSTWKVGVINNIGDTSVRLSVGRFEDLKVIIDHFEKYPLITQKLGDYKLFKQAFSVMENKEHLKENGIKELVRIKAKMNWGLNDELKKAFPENISKERPLINKNIPNLKWLAGFTSGDGNFYVHLKKSGRTTRVYVQLRFSIAQHIRDKNLMNSLITYLGCGYINEWNASERSALEFRVTKFSDINDKIIPVFQENTLIGVKLEDFEDWCKVAKLIEEKKHLTESGLDEIKKIKLNMNKGR

SEQ ID NO: 23 - protein, 909 aa, Artificial Sequence
  Synthesized megaTAL PD-1.IgV.exon2_RD1_PS3
MGSAPPKKKRKVVDLRTLGYSQQQQEKIKPKVRSTVAQHHEALVGHGFTHAHIVALSQHPAALGTVAVTYQHIITALPEATHEDIVGVGKQWSGARALEALLTDAGELRGPPLQLDTGQLVKIAKRGGVTAMEAVHASRNALTGAPLNLTPDQVVAIASNNGGKQALETVQRLLPVLCQDHGLTPDQVVAIASNGGGKQALETVQRLLPVLCQDHGLTPDQVVAIASHDGGKQALETVQRLLPVLCQDHGLTPDQVVAIASNIGGKQALETVQRLLPVLCQDHGLTPDQVVAIASHDGGKQALETVQRLLPVLCQDHGLTPDQVVAIASNIGGKQALETVQRLLPVLCQDHGLTPDQVVAIASHDGGKQALETVQRLLPVLCQDHGLTPDQVVAIASNIGGKQALETVQRLLPVLCQDHGLTPDQVVAIASNIGGKQALETVQRLLPVLCQDHGLTPDQVVAIASHDGGKQALETVQRLLPVLCQDHGLTPDQVVAIASNGGGKQALETVQRLLPVLCQDHGLTPDQVVAIASNNGGKQALESIVAQLSRPDPALAALTNDHLVALACLGGRPAMDAVKKGLPHAPELIRRVNRRIGERTSHRVAISRVGGSSRRESINPWILTGFADAEGCFLLHIRNLNRTSTKYRTRLSFEIELHNKDKSILENIQSTWKVGIINNIGNRRVRLSVRRFEDLKVIIDHFEKYPLITQKLGDYKLFKQAFSLMENKEHLKENGIKELVRIKAKMNWGLNDELKKAFPENISKERPLINKNIPNLKWLAGFTSGDGNFYVHLKKSGRTTRVYVQLRFSISQHIRDKNLMNSLITYLGCGYITESNPSERSDLEFRVTKFSDINDKIIPVFQENTLIGVKLEDFEDWCKVAKLIEEKKHLTESGLDEIKKIKLNMNKGR

SEQ ID NO: 24 - protein, 236 aa, Mus musculus
MSEPPRAETFVFLDLEATGLPNMDPEIAEISLFAVHRSSLENPERDDSGSLVLPRVLDKLTLCMCPERPFTAKASEITGLSSESLMHCGKAGFNGAVVRTLQGFLSRQEGPICLVAHNGFDYDFPLLCTGLQRLGAHLPQDTVCLDTLPALRGLDRAHSHGTRAQGRKSYSLASLFHRYFQAEPSAAHSAEGDVHTLLLIFLHRAPELLAWADEQARSWAHIEPMYVPPDGPSLEA

SEQ ID NO: 25 - DNA, 22 bp, Homo sapiens
aatggtggcatactccgtctgc

SEQ ID NO: 26 - DNA, 11 bp, Homo sapiens
tccgctaggaa

SEQ ID NO: 27 - DNA, 37 bp, Homo sapiens
tccgctaggaaagacaatggtggcatactccgtctgc

SEQ ID NO: 28 - DNA, 22 bp, Homo sapiens
aatggtggcatacaacctttta

SEQ ID NO: 29 - DNA, 22 bp, Homo sapiens
tttccacttatactccgtctgc

SEQ ID NO: 30 - DNA, 22 bp, Homo sapiens
ggcatgcagatcccacaggcgc

SEQ ID NO: 31 - DNA, 14 bp, Homo sapiens
ggtggggctgctcc

SEQ ID NO: 32 - DNA, 37 bp, Homo sapiens
ggtggggctgctccaggcatgcagatcccacaggcgc

SEQ ID NO: 33 - DNA, 22 bp, Homo sapiens
ggcatgcagatccaacctttta

SEQ ID NO: 34 - DNA, 22 bp, Homo sapiens
tttccacttatcccacaggcgc

SEQ ID NO: 35 - DNA, 22 bp, Homo sapiens
acgggcgtgacttccacatgag

SEQ ID NO: 36 - DNA, 12 bp, Homo sapiens
gtcacacaactg

SEQ ID NO: 37 - DNA, 38 bp, Homo sapiens
gtcacacaactgcccaacgggcgtgacttccacatgag

SEQ ID NO: 38 - DNA, 22 bp, Homo sapiens
acgggcgtgacttaacctttta

SEQ ID NO: 39 - DNA, 22 bp, Homo sapiens
tttccacttacttccacatgag

SEQ ID NO: 40 - RNA, 2650 nt, Artificial Sequence
  Synthesized PD-1 Exon5 RD5_CV23MK megaTAL mRNA
augggauccgccccccccaagaagaagcgcaaggugguggaccugagaacccugggguacagccagcagcaacaggagaagaucaaaccgaaggugcgcagcacgguggcccagcaccaugaagcccucgugggucauggauucacgcacgcccacaucguggcccugucgcagcauccggccgcccugggcaccguggcggugaccuaccagcacaucaucaccgcccugcccgaagccacccacgaggacaucgugggagugggcaagcagugguccggagcacgcgcccuggaggcccugcugaccgacgccggggaacugcgcggcccgccucugcagcuggauaccggccaacuggucaagaucgccaagagaggcggagugaccgcgauggaggccguccacgccucccggaacgcucugaccggugccccgcucaaucugacuccggaccaggugguggcuaucgccagcaacggaggaggaaaacaggcccucgaaacagugcagaggcugcugccuguccuuugucaagaucacgggcugacucccgaccaggucguggccauugccagccacgacggcggcaagcaggcuuuggagacugugcagcggcuccugccagugcugugccaagaucacggucugaccccagaucaggucgucgccauugcuuccaacggaggcaaacaagcgcuggaaacgguccaacgccugcugccggugcuuugucaggaucacggccugaccccugaucaggugguggccaucgcguccaauaacggggggaagcaggcacucgagacuguccagaggcuccugccugugcucugccaggaccacgggcucacacccgaucaggucgucgcuaucgcgucgcacgacgguggaaagcaggcccuggaaaccgugcagcgccuguugccggugcugugucaggaccauggccuuacuccggaucaggucgucgcgaucgcaucuaaugguggaggaaagcaggcccuggagacaguccagcgccugcucccgguguugugccaagaccauggucuuaccccugaccagguggucgcuauugccucgaacaucggcggaaagcaagcccuggaaaccgugcagcgacuucugccgguccugugccaggaucauggauugaccccagaccaggugguggcgauugccagcaacaacggcgggaagcaagcguuggaaaccguccagagacugcuuccugugcugugccaagaccacgguuugaccccggaccaagucgucgccaucgcuuccaacaacggagggaagcaggcacucgaaacugugcaacgguugcugcccgugcucugucaggaucacggacucaccccugaucaggugguggccaucgcaagcaacaucgguggcaaacaggcucuggaaacuguccaaagacugcugcccgugcuuugccaggaccacggacugacuccugaccaagugguggcaauugccuccaacaucggaggcaagcaagcgcucgaauccaucguggcgcagcucagccggccagaccccgcccuggccgcccugacuaacgaucaccugguggcccuggcgugccucggcggucgccccgcuauggacgcggugaagaaggggcugccccacgcccccgagcucauucggcgggugaaccgccggaucggagaaagaaccucccaucggguggccaucucgagaucacggcgggaauccauuaaccccuggauccugacuggcuuugccgacgccgagggauccuuccagcucgaaauccggaacgugaacccaaacaucccccgguaucgcaccagacugcgguucgagaucgaccuucacaacaaggacaaguccauucuggaggacauccagucaaccuggaaagugggaaagaucuacaaccagggggacucauacgugaagcugcgggugacccgcuucgaagaucucaaagugaucaucgaccauuucgagaaguacccccugaucacucagaagcuuggagacuacaaacuguucaagcaggcauucuccgugauggagaacaaggagcaccugaaggagaacgggauuaaggagcuggugcgaauuaaggcgaaaaugaacuggggauugaacgaugagcugaagaaggcguucccggaaaacauuuccaaggagcgcccgcucaucaacaagaacaucccuaaucugaaguggcucgcgggguuuaccucuggcgacggccauuucggagugauucucgcaaagcgcaggcccgccagcccugugcaagugcggcugcgguucaugaucggccagcacauuaaggacaagaaccugaugaacucgcucaucaccuaccuuggaugcggccggauucgcgaaaagaacaagagcgagaaguccuggcuggaauuugaagugaccaaguucagcgacaucaacgacaagaucauuccgguguuccaggaaaacacccugauuggcgugaagcuggaggacuucgaggauuggugcaagguggccaagcucaucgaagaaaagaagcaccugacugaauccggcuuggacgagaucaagaagauuaagcugaauaugaacaagggaaggugauagcgcgcuagccguacggaaaaaaaaaaaaaaaaaa

SEQ ID NO: 41 - RNA, 2526 nt, Artificial Sequence
  Synthesized PD-1 Exon1 RD2_B1H8 megaTAL mRNA
augggaagcgccccgccgaagaagaagcgcaaggugguggaucugagaacccugggauacagccagcagcagcaggagaagaucaagccgaagguccggucuaccguggcccagcaccaugaggcccuugugggccacggcuucacacaugcacacaucgucgcccugucgcagcaucccgccgcccuggggaccguggccgugaccuaucaacacaucauuaccgcccugccggaggccacccacgaggacaucguggguguggggaagcaguggagcggagccagggcacucgaagcccuccucacugacgcuggagaacugcgcggaccgccucuccagcuggacaccggacagcuggugaaaaucgccaagcggggaggagugaccgccauggaagccgugcacgccucgaggaacgcgcugacuggcgccccucugaaccugaccccugaucaggucguggcuaucgccucaaacaacggggguaagcaggcgcuggagacagugcaacgacuucugccagugcuuugucaggaccauggucugacccccgaccaggucgucgccauugcauccaacaaugguggcaagcaggcacuggagacuguccagaggcugcucccggugcugugccaggaccacgggcucaccccggaccaaguggucgccaucgccuccaacggaggaggaaaacaagcucuggagacugugcaacgccugcugccuguguugugccaagaccacggacugacgcccgaucaggugguggcgaucgcaucgaacaacggaggaaagcaagcgcuggaaaccgugcagcgccuccugcccguccucugccaggaucacggccugacuccggaccagguggucgcgaucgccagcaauaacggggggaagcaagcccucgagacugugcagcgguugcugcccgugcucugccaagaucauggccuuaccccagaccaagucguggccauugcuuccaacaacgguggcaaacaggcgcucgaaaccguccagcggcuguugcccgugcuuugccaggaucacggacucaccccugaucaggugguggcaauugcguccaacaacgguggaaagcaggcccuggaaacggugcagcggcugcuuccgguccugugucaggaucaugggcugacucccgaccaggucgucgccauugcaucccacgauggggguaaacaggcccucgaaacagugcagagacuccugccaguccugugccaagaccacggacuuaccccggaucaggugguggccauagccucgaacggcggcgggaaacaggcucuggaaacugugcaaagacuccucccgguguugugucaagaccauggacugaccccagaucaggugguggcuauugccucuaacaacggcggcaagcaagcacucgaaagcaucguggcccaguugucacgccccgaccccgcacuggcugcccugacgaaugaccaucugguggcgcuggccugccugggagggaggccagcgauggaugcggugaagaagggacugccccaugcuccggagcugauucggagagugaauaggcgcaucggagagagaacuucacaucggguggccauuucuagagugggcggcagcucccggcgcgaguccauuaaccccuggauccugaccggcuuugccgacgccgaaggguccuucggccucucgauccugaaccggaaccgggguaccgcucgguaccacaccagacuguccuucaccaucgugcugcacaacaaggacaagagcauccucgaaaacauucagucaacguggaaggugggaauuauuacuaacgacggcgacagauacgugcgccugugcgugacccgguuugaggaccugaaggucauuaucgaccacuucgagaaguacccccucgugacucagaagcugggagacuacaagcuguucaagcaggcguucucggugauggaaaacaaggagcaccugaaggagaacggcaucaaggagcucgcccggaucaaggccaagaugaacuggggccugaaugaugaacucaagaaggcguucccugaaaacaucgguaaagaacggccccugaucaacaagaacaucccgaacuucaaguggcuugccggauucaccuccggcgacggauccuucuucguccggcugcgcaaguccaacgugaacgcgagagugcgggugcaauuggucuuugaaaucucacagcacaucagggacaagaauuugaugaacucccucaucaccuaccuggguugcggacacaucuacgaaggcaauaagucggagcggagcuggcugcaguuucgcguggaaaaguucuccgacauuaacgacaagaucaucccaguguuccaggaaaacacucugauuggcgugaagcuugaggauuucgaggacuggugcaagguggccaagcugauugaagagaagaagcaccugaccgaguccggccuggacgaaaucaagaaaaucaagcugaacaugaacaagggacgguga

SEQ ID NO: 42 - RNA, 2730 nt, Artificial Sequence
  Synthesized PD-1 Exon2 RD1_G5 megaTAL mRNA
augggaagcgccccuccgaagaagaagcgcaaggucguggaccucagaacccuggguuacucccagcagcagcaggagaaaauuaagccgaaggugcgcuccaccguggcucaacaccacgaggcccucgugggccauggauucacucacgcccauaucguggcccugucccagcacccggccgcccugggcaccguggcggugaccuaccagcacaucaucaccgcgcugccugaagccacccacgaggacaucgucgguguggguaagcagugguccggagccagagcccuggaggcucugcugaccgacgccggagaacucagaggcccgccucugcagcuggacaccggacagcuggugaagauagccaagagaggcggcgugaccgccauggaagccgugcaugcgucccgcaacgcacugaccggggccccccugaaccugacuccagaccaagugguggcuaucgccagcaacaauggaggaaagcaagccuuggaaaccgugcagcggcugcucccgguccuuugccaagaccacggccugacacccgaucaggugguggcaaucgcaucgaauggcggcgggaagcaggcccucgagacugugcagaggcuccugccugugcugugccaggaccaugggcugaccccagaccagguggucgcaaucgccucgcacgacggaggcaagcaagcccuggaaacuguccagcgccugcucccuguccugugucaagaucaugggcucacuccugaucaggucgucgccaucgccucgaacauugguggcaagcaggcgcucgaaaccguccagcgguugcugccagugcuuugccaggaccauggucugacccccgaucaaguggucgcgauugccucacacgauggcgguaagcaggcuuuggaaaccgugcaacggcuguugccuguccucugccaggaccacggcuugacucccgaccaggugguggccauagccucaaacaucggagggaaacaagcccucgaaaccguccagaggcugcugccgguguugugccaggaucacggauugaccccagaccagguggucgccauugcuucccacgaugggggaaagcaggcccuggagacugugcagcgccuccuucccguccugugucaggaucauggacuuacccccgaccaagucguggcgauugcuuccaauaucggaggcaaacaggcccuugaaacagugcagcgccuguugccggugcucugccaagaucacggacugaccccugaccaggugguggcgaucgcgucaaauaucggcggcaagcaggcacuggagacaguccagagacuccugccgguccucugccaggaccacggucuuacuccugaccaagugguggcuaucgcaucccaugauggugggaaacaggcucuugaaacugugcaacgccugcugcccgugcugugccaagaccacggacugacuccggaccaggucguggccaucgcuucaaacggagggggaaaacaggcacuugaaacggugcagagacugcugccuguccuuugucaggaccacggguugaccccggaccaggucguggcuauugccucgaacaacggggggaagcaagcgcucgaguccauuguggcccagcugagccggccugaucccgcacuggccgcgcugaccaacgaucaccugguggcccucgccugucugggcggacggccggccauggacgccgugaagaagggacugccgcacgcgcccgagcugauccgccgcgugaacaggcggauuggagaacgcaccucccaccggguggccaucucgagagugggaggauccucuagacgggaguccauuaacccguggauccugacuggauucgccgacgccgagggguccuuccagcuguacaucuccaacgugaacaacaaccgcagcagauacagggcccggcugcgguucgcgaucgaacugcacaauaaggacaagagcauccucgagaacauucaguccacuuggaaggugggcgugauuaacaacaucggcgauaccagcgugcggcucuccguggggcgguucgaagaucucaaggugaucaucgaccacuucgagaaguacccgcugaucacccagaagcugggagacuacaagcuguucaagcaagcuuucagcgugauggaaaacaaggaacaucugaaagagaacgguaucaaggaacuggugcggauuaaggccaagaugaacuggggucugaacgaugaacugaagaaggcguucccggagaauaucagcaaggagcgcccccugauuaacaaaaacaucccaaaccucaaguggcucgccggcuuuacuuccggagaugguaacuucuacgugcaccugaagaaguccggaagaaccacccgggucuacgugcagcugagguucuccaucgcccagcacauccgggacaagaacuugaugaacucccugaucaccuaccucgguugcggauacaucaacgaauggaacgccagcgagagaucggcccuggaguucagggugacuaaguucuccgacaucaacgacaagauuauccccguguuucaggaaaauacccucaucggcgugaagcuggaggacuuugaggacuggugcaagguggccaagcugaucgaggaaaagaaacaucugaccgagagcggccuggacgaaaucaagaagauuaagcugaacaugaacaagggacgauga

SEQ ID NO: 43 - RNA, 711 nt, Mus musculus
augucugagccaccucgggcugagaccuuuguauuccuggaccuagaagccacugggcucccaaacauggacccugagauugcagagauaucccuuuuugcuguucaccgcucuucccuggagaacccagaacgggaugauucugguuccuuggugcugccccguguucuggacaagcucacacugugcaugugcccggagcgccccuuuacugccaaggccagugagauuacugguuugagcagcgaaagccugaugcacugcgggaaggcugguuucaauggcgcugugguaaggacacugcagggcuuccuaagccgccaggagggccccaucugccuuguggcccacaauggcuucgauuaugacuucccacugcugugcacggggcuacaacgucugggugcccaucugccccaagacacugucugccuggacacacugccugcauugcggggccuggaccgugcucacagccacggcaccagggcucaaggccgcaaaagcuacagccuggccagucucuuccaccgcuacuuccaggcugaacccagugcugcccauucagcagaaggugaugugcacacccugcuucugaucuuccugcaucgugcuccugagcugcucgccugggcagaugagcaggcccgcagcugggcucauauugagcccauguacgugccaccugaugguccaagccucgaagccuga

SEQ ID NO: 44 - DNA, 7601 bp, Artificial Sequence
  Synthesized rAAV PD-1 Exon5_MND-BFP construct
cagctgcgcgctcgctcgctcactgaggccgcccgggcaaagcccgggcgtcgggcgacctttggtcgcccggcctcagtgagcgagcgagcgcgcagagagggagtggccaactccatcactaggggttccttgtagttaatgattaacccgccatgctacttatctacgtagaattcagtccagggctctgtcctgcacctggggaatggtgaccggcatctctgtcctctagctctggaagcaccccagcccctctagtctgccctcacccctgaccctgaccctccaccctgaccccgtcctaacccctgacctttgtgcccttccagagagaagggcagaagtgcccacagcccaccccagcccctcacccaggccagccggccagttccaaaccctggtggttggtgtcgtgggcggcctgctgggcagcctggtgctgctagtctgggtcctggccgtcatctgctcccgggccgcacgaggtaacgtcatcccagcccctcggcctgccctgccctaaccctgctggcggccctcactcccgcctccccttcctccacccttccctcaccccaccccacctccccccatctccccgccaggctaagtccctgatgaaggcccctggactaagaccccccacctaggagcacggctcagggtcggcctggtgaccccaagtgtgtttctctgcagggacaataggagccaggcgcaccggccagcccctggtgagtctcactcttttcctgcatgatccactgtgccttccttcctgggtgggcagaggtggaaggacaggctgggaccacacggcctgcaggactcacattctattatagccaggaccccacctccccagcccccaggcagcaacctcaatccctaaagccatgatctggggccccagcccacctgcggtctccgggggtgcccggcccatgtgtgtgcctgcctgcggtctccaggggtgcctggcccacgcgtgtgcccgcctgcggtctctgggggtgcccggcccacatatgtgcctgcctgcggtctccaggtgtgcccggcccatgcgtgtgcccacctgcgagggcgtggggtgggcttggtcatttcttatcttacattggagacaggagagcttgaaaagtcacattttggaatcctaaatctgcaagaatgccagggacatttcagagggggacattgagccagagaggaggggtggtgtccccagatcacacagagggcagtggtgggacagctcagggtaagcagctcatagtggggggcccaggttcggtgccggtactgcagccaggctgtggagccgcgggcctccttcctgcggtgggccgtggggctgactccctctccctttctcctcaaagaaggaggacccctcagccgtgcctgtgttctctgtggactatggggagctggatttccagtggcgagagaagaccccggagccccccgtgccctgtgtccctgagcagacggagtaatgcatgaacagagaaacaggagaatatgggccaaacaggatatctgtggtaagcagttcctgccccggctcagggccaagaacagttggaacagcagaatatgggccaaacaggatatctgtggtaagcagttcctgccccggctcagggccaagaacagatggtccccagatgcggtcccgccctcagcagtttctagagaaccatcagatgtttccagggtgccccaaggacctgaaatgaccctgtgccttatttgaactaaccaatcagttcgcttctcgcttctgttcgcgcgcttctgctccccgagctctatataagcagagctcgtttagtgaaccgtcagatcgcctggagacgccatccacgctgttttgacttccatagaaggatctcgaggccaccatggctagcgagctgattaaggagaacatgcacatgaagctgtacatggagggcaccgtggacaaccatcacttcaagtgcacatccgagggcgaaggcaagccctacgagggcacccagaccatgagaatcaaggtggtcgagggcggccctctccccttcgccttcgacatcctggctactagcttcctctacggcagcaagaccttcatcaaccacacccagggcatccccgacttcttcaagcagtccttccctgagggcttcacatgggagagagtcaccacatacgaggacgggggcgtgctgaccgctacccaggacaccagcctccaggacggctgcctcatctacaacgtcaagatcagaggggtgaacttcacatccaacggccctgtgatgcagaagaaaacactcggctgggaggccttcaccgagacgctgtaccccgctgacggcggcctggaaggcagaaacgacatggccctgaagctcgtgggcgggagccatctgatcgcaaacatcaagaccacatatagatccaagaaacccgctaagaacctcaagatgcctggcgtctactatgtggactacagactggaaagaatcaaggaggccaacaacgagacctacgtcgagcagcacgaggtggcagtggccagatactgcgacctccctagcaaactggggcacaagctaaattgaaagctttgctttatttgtgaaatttgtgatgctattgctttatttgtaaccattataagctgcaataaacaagtttaacaacaacaattgcattcattttatgtttcaggttcagggggaggtgtgggaggttttttaaagtcgacccaccattgtctttcctagcggaatgggcacctcatcccccgcccgcaggggctcagctgacggccctcggagtgcccagccactgaggcctgaggatggacactgctcttggcccctctgaccggcttccttggccaccagtgttctgcagaccctccaccatgagcccgggtcagcgcatttcctcaggagaagcaggcagggtgcaggccattgcaggccgtccaggggctgagctgcctgggggcgaccggggctccagcctgcacctgcaccaggcacagccccaccacaggactcatgtctcaatgcccacagtgagcccaggcagcaggtgtcaccgtcccctacagggagggccagatgcagtcactgcttcaggtcctgccagcacagagctgcctgcgtccagctccctgaatctctgctgctgctgctgctgctgctgctgctgcctgcggcccggggctgaaggcgccgtggccctgcctgacgccccggagcctcctgcctgaacttgggggctggttggagatggccttggagcagccaaggtgcccctggcagtggcatcccgaaacgccctggacgcagggcccaagactgggcacaggagtgggaggtacatggggctggggactccccaggagttatctgctccctgcaggcctagagaagtttcagggaaggtcagaagagctcctggctgtggtgggcagggcaggaaacccctccacctttacacatgcccaggcagcacctcaggccctttgtggggcagggaagctgaggcagtaagcgggcaggcagagctggaggcctttcaggcccagccagcactctggcctcctgccgccgcattccaccccagcccctcacaccactcgggagagggacatcctacggtcccaaggtcaggagggcagggctggggttgactcaggcccctcccagctgtggccacctgggtgttgggagggcagaagtgcaggcacctagggccccccatgtgcccaccctgggagctctccttggaacccattcctgaaattatttaaaggggttggccggactagttacgtagataagtagcatggcgggttaatcattaactacaaggaacccctagtgatggagttggccactccctctctgcgcgctcgctcgctcactgaggccgggcgaccaaaggtcgcccgacgcccgggctttgcccgggcggcctcagtgagcgagcgagcgcgccagctggcgtaatagcgaagaggcccgcaccgatcgcccttcccaacagttgcgcagcctgaatggcgaatggcgattccgttgcaatggctggcggtaatattgttctggatattaccagcaaggccgatagtttgagttcttctactcaggcaagtgatgttattactaatcaaagaagtattgcgacaacggttaatttgcgtgatggacagactcttttactcggtggcctcactgattataaaaacacttctcaggattctggcgtaccgttcctgtctaaaatccctttaatcggcctcctgtttagctcccgctctgattctaacgaggaaagcacgttatacgtgctcgtcaaagcaaccatagtacgcgccctgtagcggcgcattaagcgcggcgggtgtggtggttacgcgcagcgtgaccgctacacttgccagcgccctagcgcccgctcctttcgctttcttcccttcctttctcgccacgttcgccggctttccccgtcaagctctaaatcgggggctccctttagggttccgatttagtgctttacggcacctcgaccccaaaaaacttgattagggtgatggttcacgtagtgggccatcgccctgatagacggtttttcgccctttgacgttggagtccacgttctttaatagtggactcttgttccaaactggaacaacactcaaccctatctcggtctattcttttgatttataagggattttgccgatttcggcctattggttaaaaaatgagctgatttaacaaaaatttaacgcgaattttaacaaaatattaacgtttacaatttaaatatttgcttatacaatcttcctgtttttggggcttttctgattatcaaccggggtacatatgattgacatgctagttttacgattaccgttcatcgattctcttgtttgctccagactctcaggcaatgacctgatagcctttgtagagacctctcaaaaatagctaccctctccggcatgaatttatcagctagaacggttgaatatcatattgatggtgatttgactgtctccggcctttctcacccgtttgaatctttacctacacattactcaggcattgcatttaaaatatatgagggttctaaaaatttttatccttgcgttgaaataaaggcttctcccgcaaaagtattacagggtcataatgtttttggtacaaccgatttagctttatgctctgaggctttattgcttaattttgctaattctttgccttgcctgtatgatttattggatgttggaatcgcctgatgcggtattttctccttacgcatctgtgcggtatttcacaccgcatatggtgcactctcagtacaatctgctctgatgccgcatagttaagccagccccgacacccgccaacacccgctgacgcgccctgacgggcttgtctgctcccggcatccgcttacagacaagctgtgaccgtctccgggagctgcatgtgtcagaggttttcaccgtcatcaccgaaacgcgcgagacgaaagggcctcgtgatacgcctatttttataggttaatgtcatgataataatggtttcttagacgtcaggtggcacttttcggggaaatgtgcgcggaacccctatttgtttatttttctaaatacattcaaatatgtatccgctcatgagacaataaccctgataaatgcttcaataatattgaaaaaggaagagtatgagtattcaacatttccgtgtcgcccttattcccttttttgcggcattttgccttcctgtttttgctcacccagaaacgctggtgaaagtaaaagatgctgaagatcagttgggtgcacgagtgggttacatcgaactggatctcaacagcggtaagatccttgagagttttcgccccgaagaacgttttccaatgatgagcacttttaaagttctgctatgtggcgcggtattatcccgtattgacgccgggcaagagcaactcggtcgccgcatacactattctcagaatgacttggttgagtactcaccagtcacagaaaagcatcttacggatggcatgacagtaagagaattatgcagtgctgccataaccatgagtgataacactgcggccaacttacttctgacaacgatcggaggaccgaaggagctaaccgcttttttgcacaacatgggggatcatgtaactcgccttgatcgttgggaaccggagctgaatgaagccataccaaacgacgagcgtgacaccacgatgcctgtagcaatggcaacaacgttgcgcaaactattaactggcgaactacttactctagcttcccggcaacaattaatagactggatggaggcggataaagttgcaggaccacttctgcgctcggcccttccggctggctggtttattgctgataaatctggagccggtgagcgtgggtctcgcggtatcattgcagcactggggccagatggtaagccctcccgtatcgtagttatctacacgacggggagtcaggcaactatggatgaacgaaatagacagatcgctgagataggtgcctcactgattaagcattggtaactgtcagaccaagtttactcatatatactttagattgatttaaaacttcatttttaatttaaaaggatctaggtgaagatcctttttgataatctcatgaccaaaatcccttaacgtgagttttcgttccactgagcgtcagaccccgtagaaaagatcaaaggatcttcttgagatcctttttttctgcgcgtaatctgctgcttgcaaacaaaaaaaccaccgctaccagcggtggtttgtttgccggatcaagagctaccaactctttttccgaaggtaactggcttcagcagagcgcagataccaaatactgtccttctagtgtagccgtagttaggccaccacttcaagaactctgtagcaccgcctacatacctcgctctgctaatcctgttaccagtggctgctgccagtggcgataagtcgtgtcttaccgggttggactcaagacgatagttaccggataaggcgcagcggtcgggctgaacggggggttcgtgcacacagcccagcttggagcgaacgacctacaccgaactgagatacctacagcgtgagctatgagaaagcgccacgcttcccgaagggagaaaggcggacaggtatccggtaagcggcagggtcggaacaggagagcgcacgagggagcttccagggggaaacgcctggtatctttatagtcctgtcgggtttcgccacctctgacttgagcgtcgatttttgtgatgctcgtcaggggggcggagcctatggaaaaacgccagcaacgcggcctttttacggttcctggccttttgctggccttttgctcacatgttctttcctgcgttatcccctgattctgtggataaccgtattaccgcctttgagtgagctgataccgctcgccgcagccgaacgaccgagcgcagcgagtcagtgagcgaggaagcggaagagcgcccaatacgcaaaccgcctctccccgcgcgttggccgattcattaatg

SEQ ID NO: 45 - DNA, 1325 bp, Homo sapiens
agtccagggctctgtcctgcacctggggaatggtgaccggcatctctgtcctctagctctggaagcaccccagcccctctagtctgccctcacccctgaccctgaccctccaccctgaccccgtcctaacccctgacctttgtgcccttccagagagaagggcagaagtgcccacagcccaccccagcccctcacccaggccagccggccagttccaaaccctggtggttggtgtcgtgggcggcctgctgggcagcctggtgctgctagtctgggtcctggccgtcatctgctcccgggccgcacgaggtaacgtcatcccagcccctcggcctgccctgccctaaccctgctggcggccctcactcccgcctccccttcctccacccttccctcaccccaccccacctccccccatctccccgccaggctaagtccctgatgaaggcccctggactaagaccccccacctaggagcacggctcagggtcggcctggtgaccccaagtgtgtttctctgcagggacaataggagccaggcgcaccggccagcccctggtgagtctcactcttttcctgcatgatccactgtgccttccttcctgggtgggcagaggtggaaggacaggctgggaccacacggcctgcaggactcacattctattatagccaggaccccacctccccagcccccaggcagcaacctcaatccctaaagccatgatctggggccccagcccacctgcggtctccgggggtgcccggcccatgtgtgtgcctgcctgcggtctccaggggtgcctggcccacgcgtgtgcccgcctgcggtctctgggggtgcccggcccacatatgtgcctgcctgcggtctccaggtgtgcccggcccatgcgtgtgcccacctgcgagggcgtggggtgggcttggtcatttcttatcttacattggagacaggagagcttgaaaagtcacattttggaatcctaaatctgcaagaatgccagggacatttcagagggggacattgagccagagaggaggggtggtgtccccagatcacacagagggcagtggtgggacagctcagggtaagcagctcatagtggggggcccaggttcggtgccggtactgcagccaggctgtggagccgcgggcctccttcctgcggtgggccgtggggctgactccctctccctttctcctcaaagaaggaggacccctcagccgtgcctgtgttctctgtggactatggggagctggatttccagtggcgagagaagaccccggagccccccgtgccctgtgtccctgagcagacggagta

SEQ ID NO: 46 - DNA, 1072 bp, Homo sapiens
ccaccattgtctttcctagcggaatgggcacctcatcccccgcccgcaggggctcagctgacggccctcggagtgcccagccactgaggcctgaggatggacactgctcttggcccctctgaccggcttccttggccaccagtgttctgcagaccctccaccatgagcccgggtcagcgcatttcctcaggagaagcaggcagggtgcaggccattgcaggccgtccaggggctgagctgcctgggggcgaccggggctccagcctgcacctgcaccaggcacagccccaccacaggactcatgtctcaatgcccacagtgagcccaggcagcaggtgtcaccgtcccctacagggagggccagatgcagtcactgcttcaggtcctgccagcacagagctgcctgcgtccagctccctgaatctctgctgctgctgctgctgctgctgctgctgcctgcggcccggggctgaaggcgccgtggccctgcctgacgccccggagcctcctgcctgaacttgggggctggttggagatggccttggagcagccaaggtgcccctggcagtggcatcccgaaacgccctggacgcagggcccaagactgggcacaggagtgggaggtacatggggctggggactccccaggagttatctgctccctgcaggcctagagaagtttcagggaaggtcagaagagctcctggctgtggtgggcagggcaggaaacccctccacctttacacatgcccaggcagcacctcaggccctttgtggggcagggaagctgaggcagtaagcgggcaggcagagctggaggcctttcaggcccagccagcactctggcctcctgccgccgcattccaccccagcccctcacaccactcgggagagggacatcctacggtcccaaggtcaggagggcagggctggggttgactcaggcccctcccagctgtggccacctgggtgttgggagggcagaagtgcaggcacctagggccccccatgtgcccaccctgggagctctccttggaacccattcctgaaattatttaaaggggttggccgg

SEQ ID NO: 47 - DNA, 7601 bp, Artificial Sequence
  Synthesized rAAV PD-1 Exon5_MND-BFP 3'-Homology Arm SNP construct
cagctgcgcgctcgctcgctcactgaggccgcccgggcaaagcccgggcgtcgggcgacctttggtcgcccggcctcagtgagcgagcgagcgcgcagagagggagtggccaactccatcactaggggttccttgtagttaatgattaacccgccatgctacttatctacgtagaattcagtccagggctctgtcctgcacctggggaatggtgaccggcatctctgtcctctagctctggaagcaccccagcccctctagtctgccctcacccctgaccctgaccctccaccctgaccccgtcctaacccctgacctttgtgcccttccagagagaagggcagaagtgcccacagcccaccccagcccctcacccaggccagccggccagttccaaaccctggtggttggtgtcgtgggcggcctgctgggcagcctggtgctgctagtctgggtcctggccgtcatctgctcccgggccgcacgaggtaacgtcatcccagcccctcggcctgccctgccctaaccctgctggcggccctcactcccgcctccccttcctccacccttccctcaccccaccccacctccccccatctccccgccaggctaagtccctgatgaaggcccctggactaagaccccccacctaggagcacggctcagggtcggcctggtgaccccaagtgtgtttctctgcagggacaataggagccaggcgcaccggccagcccctggtgagtctcactcttttcctgcatgatccactgtgccttccttcctgggtgggcagaggtggaaggacaggctgggaccacacggcctgcaggactcacattctattatagccaggaccccacctccccagcccccaggcagcaacctcaatccctaaagccatgatctggggccccagcccacctgcggtctccgggggtgcccggcccatgtgtgtgcctgcctgcggtctccaggggtgcctggcccacgcgtgtgcccgcctgcggtctctgggggtgcccggcccacatatgtgcctgcctgcggtctccaggtgtgcccggcccatgcgtgtgcccacctgcgagggcgtggggtgggcttggtcatttcttatcttacattggagacaggagagcttgaaaagtcacattttggaatcctaaatctgcaagaatgccagggacatttcagagggggacattgagccagagaggaggggtggtgtccccagatcacacagagggcagtggtgggacagctcagggtaagcagctcatagtggggggcccaggttcggtgccggtactgcagccaggctgtggagccgcgggcctccttcctgcggtgggccgtggggctgactccctctccctttctcctcaaagaaggaggacccctcagccgtgcctgtgttctctgtggactatggggagctggatttccagtggcgagagaagaccccggagccccccgtgccctgtgtccctgagcagacggagtaatgcatgaacagagaaacaggagaatatgggccaaacaggatatctgtggtaagcagttcctgccccggctcagggccaagaacagttggaacagcagaatatgggccaaacaggatatctgtggtaagcagttcctgccccggctcagggccaagaacagatggtccccagatgcggtcccgccctcagcagtttctagagaaccatcagatgtttccagggtgccccaaggacctgaaatgaccctgtgccttatttgaactaaccaatcagttcgcttctcgcttctgttcgcgcgcttctgctccccgagctctatataagcagagctcgtttagtgaaccgtcagatcgcctggagacgccatccacgctgttttgacttccatagaaggatctcgaggccaccatggctagcgagctgattaaggagaacatgcacatgaagctgtacatggagggcaccgtggacaaccatcacttcaagtgcacatccgagggcgaaggcaagccctacgagggcacccagaccatgagaatcaaggtggtcgagggcggccctctccccttcgccttcgacatcctggctactagcttcctctacggcagcaagaccttcatcaaccacacccagggcatccccgacttcttcaagcagtccttccctgagggcttcacatgggagagagtcaccacatacgaggacgggggcgtgctgaccgctacccaggacaccagcctccaggacggctgcctcatctacaacgtcaagatcagaggggtgaacttcacatccaacggccctgtgatgcagaagaaaacactcggctgggaggccttcaccgagacgctgtaccccgctgacggcggcctggaaggcagaaacgacatggccctgaagctcgtgggcgggagccatctgatcgcaaacatcaagaccacatatagatccaagaaacccgctaagaacctcaagatgcctggcgtctactatgtggactacagactggaaagaatcaaggaggccaacaacgagacctacgtcgagcagcacgaggtggcagtggccagatactgcgacctccctagcaaactggggcacaagctaaattgaaagctttgctttatttgtgaaatttgtgatgctattgctttatttgtaaccattataagctgcaataaacaagtttaacaacaacaattgcattcattttatgtttcaggttcagggggaggtgtgggaggttttttaaagtcgacccaccattgtctttcctagcggaatgggcacctcatcccccgcccgcaggggctcagccgacggccctcggagtgcccagccactgaggcctgaggatggacactgctcttggcccctctgaccggcttccttggccaccagtgttctgcagaccctccaccatgagcccgggtcagcgcatttcctcaggagaagcaggcagggtgcaggccattgcaggccgtccaggggctgagctgcctgggggcgaccggggctccagcctgcacctgcaccaggcacagccccaccacaggactcatgtctcaatgcccacagtgagcccaggcagcaggtgtcaccgtcccctacagggagggccagatgcagtcactgcttcaggtcctgccagcacagagctgcctgcgtccagctccctgaatctctgctgctgctgctgctgctgctgctgctgcctgcggcccggggctgaaggcgccgtggccctgcctgacgccccggagcctcctgcctgaacttgggggctggttggagatggccttggagcagccaaggtgcccctggcagtggcatcccgaaacgccctggacgcagggcccaagactgggcacaggagtgggaggtacatggggctggggactccccaggagttatctgctccctgcaggcctagagaagtttcagggaaggtcagaagagctcctggctgtggtgggcagggcaggaaacccctccacctttacacatgcccaggcagcacctcaggccctttgtggggcagggaagctgaggcagtaagcgggcaggcagagctggaggcctttcaggcccagccagcactctggcctcctgccgccgcattccaccccagcccctcacaccactcgggagagggacatcctacggtcccaaggtcaggagggcagggctggggttgactcaggcccctcccagctgtggccacctgggtgttgggagggcagaagtgcaggcacctagggccccccatgtgcccaccctgggagctctccttggaacccattcctgaaattatttaaaggggttggccggactagttacgtagataagtagcatggcgggttaatcattaactacaaggaacccctagtgatggagttggccactccctctctgcgcgctcgctcgctcactgaggccgggcgaccaaaggtcgcccgacgcccgggctttgcccgggcggcctcagtgagcgagcgagcgcgccagctggcgtaatagcgaagaggcccgcaccgatcgcccttcccaacagttgcgcagcctgaatggcgaatggcgattccgttgcaatggctggcggtaatattgttctggatattaccagcaaggccgatagtttgagttcttctactcaggcaagtgatgttattactaatcaaagaagtattgcgacaacggttaatttgcgtgatggacagactcttttactcggtggcctcactgattataaaaacacttctcaggattctggcgtaccgttcctgtctaaaatccctttaatcggcctcctgtttagctcccgctctgattctaacgaggaaagcacgttatacgtgctcgtcaaagcaaccatagtacgcgccctgtagcggcgcattaagcgcggcgggtgtggtggttacgcgcagcgtgaccgctacacttgccagcgccctagcgcccgctcctttcgctttcttcccttcctttctcgccacgttcgccggctttccccgtcaagctctaaatcgggggctccctttagggttccgatttagtgctttacggcacctcgaccccaaaaaacttgattagggtgatggttcacgtagtgggccatcgccctgatagacggtttttcgccctttgacgttggagtccacgttctttaatagtggactcttgttccaaactggaacaacactcaaccctatctcggtctattcttttgatttataagggattttgccgatttcggcctattggttaaaaaatgagctgatttaacaaaaatttaacgcgaattttaacaaaatattaacgtttacaatttaaatatttgcttatacaatcttcctgtttttggggcttttctgattatcaaccggggtacatatgattgacatgctagttttacgattaccgttcatcgattctcttgtttgctccagactctcaggcaatgacctgatagcctttgtagagacctctcaaaaatagctaccctctccggcatgaatttatcagctagaacggttgaatatcatattgatggtgatttgactgtctccggcctttctcacccgtttgaatctttacctacacattactcaggcattgcatttaaaatatatgagggttctaaaaatttttatccttgcgttgaaataaaggcttctcccgcaaaagtattacagggtcataatgtttttggtacaaccgatttagctttatgctctgaggctttattgcttaattttgctaattctttgccttgcctgtatgatttattggatgttggaatcgcctgatgcggtattttctccttacgcatctgtgcggtatttcacaccgcatatggtgcactctcagtacaatctgctctgatgccgcatagttaagccagccccgacacccgccaacacccgctgacgcgccctgacgggcttgtctgctcccggcatccgcttacagacaagctgtgaccgtctccgggagctgcatgtgtcagaggttttcaccgtcatcaccgaaacgcgcgagacgaaagggcctcgtgatacgcctatttttataggttaatgtcatgataataatggtttcttagacgtcaggtggcacttttcggggaaatgtgcgcggaacccctatttgtttatttttctaaatacattcaaatatgtatccgctcatgagacaataaccctgataaatgcttcaataatattgaaaaaggaagagtatgagtattcaacatttccgtgtcgcccttattcccttttttgcggcattttgccttcctgtttttgctcacccagaaacgctggtgaaagtaaaagatgctgaagatcagttgggtgcacgagtgggttacatcgaactggatctcaacagcggtaagatccttgagagttttcgccccgaagaacgttttccaatgatgagcacttttaaagttctgctatgtggcgcggtattatcccgtattgacgccgggcaagagcaactcggtcgccgcatacactattctcagaatgacttggttgagtactcaccagtcacagaaaagcatcttacggatggcatgacagtaagagaattatgcagtgctgccataaccatgagtgataacactgcggccaacttacttctgacaacgatcggaggaccgaaggagctaaccgcttttttgcacaacatgggggatcatgtaactcgccttgatcgttgggaaccggagctgaatgaagccataccaaacgacgagcgtgacaccacgatgcctgtagcaatggcaacaacgttgcgcaaactattaactggcgaactacttactctagcttcccggcaacaattaatagactggatggaggcggataaagttgcaggaccacttctgcgctcggcccttccggctggctggtttattgctgataaatctggagccggtgagcgtgggtctcgcggtatcattgcagcactggggccagatggtaagccctcccgtatcgtagttatctacacgacggggagtcaggcaactatggatgaacgaaatagacagatcgctgagataggtgcctcactgattaagcattggtaactgtcagaccaagtttactcatatatactttagattgatttaaaacttcatttttaatttaaaaggatctaggtgaagatcctttttgataatctcatgaccaaaatcccttaacgtgagttttcgttccactgagcgtcagaccccgtagaaaagatcaaaggatcttcttgagatcctttttttctgcgcgtaatctgctgcttgcaaacaaaaaaaccaccgctaccagcggtggtttgtttgccggatcaagagctaccaactctttttccgaaggtaactggcttcagcagagcgcagataccaaatactgtccttctagtgtagccgtagttaggccaccacttcaagaactctgtagcaccgcctacatacctcgctctgctaatcctgttaccagtggctgctgccagtggcgataagtcgtgtcttaccgggttggactcaagacgatagttaccggataaggcgcagcggtcgggctgaacggggggttcgtgcacacagcccagcttggagcgaacgacctacaccgaactgagatacctacagcgtgagctatgagaaagcgccacgcttcccgaagggagaaaggcggacaggtatccggtaagcggcagggtcggaacaggagagcgcacgagggagcttccagggggaaacgcctggtatctttatagtcctgtcgggtttcgccacctctgacttgagcgtcgatttttgtgatgctcgtcaggggggcggagcctatggaaaaacgccagcaacgcggcctttttacggttcctggccttttgctggccttttgctcacatgttctttcctgcgttatcccctgattctgtggataaccgtattaccgcctttgagtgagctgataccgctcgccgcagccgaacgaccgagcgcagcgagtcagtgagcgaggaagcggaagagcgcccaatacgcaaaccgcctctccccgcgcgttggccgattcattaatg

SEQ ID NO: 48 - DNA, 7601 bp, Artificial Sequence
  Synthesized rAAV PD-1 Exon5_MND-BFP 5'-Homology Arm SNP construct
cagctgcgcgctcgctcgctcactgaggccgcccgggcaaagcccgggcgtcgggcgacctttggtcgcccggcctcagtgagcgagcgagcgcgcagagagggagtggccaactccatcactaggggttccttgtagttaatgattaacccgccatgctacttatctacgtagaattcagtccagggctctgtcctgcacctggggaatggtgaccggcatctctgtcctctagctctggaagcaccccagcccctctagtctgccctcacccctgaccctgaccctccaccctgaccccgtcctaacccctgacctttgtgcccttccagagagaagggcagaagtgcccacagcccaccccagcccctcacccaggccagccggccagttccaaaccctggtggttggtgtcgtgggcggcctgctgggcagcctggtgctgctagtctgggtcctggccgtcatctgctcccgggccgcacgaggtaacgtcatcccagcccctcggcctgccctgccctaaccctgctggcggccctcactcccgcctccccttcctccacccttccctcaccccaccccacctccccccatctccccgccaggctaagtccctgatgaaggcccctggactaagaccccccacctaggagcacggctcagggtcggcctggtgaccccaagtgtgtttctctgcagggacaataggagccaggcgcaccggccagcccctggtgagtctcactcttttcctgcatgatccactgtgccttccttcctgggtgggcagaggtggaaggacaggctgggaccacacggcctgcaggactcacattctattatagccaggaccccacctccccagcccccaggcagcaacctcaatccctaaagccatgatctggggccccagcccacctgcggtctccgggggtgcccggcccatgtgtgtgcctgcctgcggtctccaggggtgcctggcccacgcgtgtgcccgcctgcggtctctgggggtgcccggcccacatatgtgcctgcctgcggtctccaggtgtgcccggcccatgcgtgtgcccacctgcgagggcgtggggtgggcttggtcatttcttatcttacattggagacaggagagcttgaaaagtcacattttggaatcctaaatctgcaagaatgccagggacatttcagagggggacattgagccagagaggaggggtggtgtccccagatcacacagagggcagtggtgggacagctcagggtaagcagctcgtagtggggggcccaggttcggtgccggtactgcagccaggctgtggagccgcgggcctccttcctgcggtgggccgtggggctgactccctctccctttctcctcaaagaaggaggacccctcagccgtgcctgtgttctctgtggactatggggagctggatttccagtggcgagagaagaccccggagccccccgtgccctgtgtccctgagcagacggagtaatgcatgaacagagaaacaggagaatatgggccaaacaggatatctgtggtaagcagttcctgccccggctcagggccaagaacagttggaacagcagaatatgggccaaacaggatatctgtggtaagcagttcctgccccggctcagggccaagaacagatggtccccagatgcggtcccgccctcagcagtttctagagaaccatcagatgtttccagggtgccccaaggacctgaaatgaccctgtgccttatttgaactaaccaatcagttcgcttctcgcttctgttcgcgcgcttctgctccccgagctctatataagcagagctcgtttagtgaaccgtcagatcgcctggagacgccatccacgctgttttgacttccatagaaggatctcgaggccaccatggctagcgagctgattaaggagaacatgcacatgaagctgtacatggagggcaccgtggacaaccatcacttcaagtgcacatccgagggcgaaggcaagccctacgagggcacccagaccatgagaatcaaggtggtcgagggcggccctctccccttcgccttcgacatcctggctactagcttcctctacggcagcaagaccttcatcaaccacacccagggcatccccgacttcttcaagcagtccttccctgagggcttcacatgggagagagtcaccacatacgaggacgggggcgtgctgaccgctacccaggacaccagcctccaggacggctgcctcatctacaacgtcaagatcagaggggtgaacttcacatccaacggccctgtgatgcagaagaaaacactcggctgggaggccttcaccgagacgctgtaccccgctgacggcggcctggaaggcagaaacgacatggccctgaagctcgtgggcgggagccatctgatcgcaaacatcaagaccacatatagatccaagaaacccgctaagaacctcaagatgcctggcgtctactatgtggactacagactggaaagaatcaaggaggccaacaacgagacctacgtcgagcagcacgaggtggcagtggccagatactgcgacctccctagcaaactggggcacaagctaaattgaaagctttgctttatttgtgaaatttgtgatgctattgctttatttgtaaccattataagctgcaataaacaagtttaacaacaacaattgcattcattttatgtttcaggttcagggggaggtgtgggaggttttttaaagtcgacccaccattgtctttcctagcggaatgggcacctcatcccccgcccgcaggggctcagctgacggccctcggagtgcccagccactgaggcctgaggatggacactgctcttggcccctctgaccggcttccttggccaccagtgttctgcagaccctccaccatgagcccgggtcagcgcatttcctcaggagaagcaggcagggtgcaggccattgcaggccgtccaggggctgagctgcctgggggcgaccggggctccagcctgcacctgcaccaggcacagccccaccacaggactcatgtctcaatgcccacagtgagcccaggcagcaggtgtcaccgtcccctacagggagggccagatgcagtcactgcttcaggtcctgccagcacagagctgcctgcgtccagctccctgaatctctgctgctgctgctgctgctgctgctgctgcctgcggcccggggctgaaggcgccgtggccctgcctgacgccccggagcctcctgcctgaacttgggggctggttggagatggccttggagcagccaaggtgcccctggcagtggcatcccgaaacgccctggacgcagggcccaagactgggcacaggagtgggaggtacatggggctggggactccccaggagttatctgctccctgcaggcctagagaagtttcagggaaggtcagaagagctcctggctgtggtgggcagggcaggaaacccctccacctttacacatgcccaggcagcacctcaggccctttgtggggcagggaagctgaggcagtaagcgggcaggcagagctggaggcctttcaggcccagccagcactctggcctcctgccgccgcattccaccccagcccctcacaccactcgggagagggacatcctacggtcccaaggtcaggagggcagggctggggttgactcaggcccctcccagctgtggccacctgggtgttgggagggcagaagtgcaggcacctagggccccccatgtgcccaccctgggagctctccttggaacccattcctgaaattatttaaaggggttggccggactagttacgtagataagtagcatggcgggttaatcattaactacaaggaacccctagtgatggagttggccactccctctctgcgcgctcgctcgctcactgaggccgggcgaccaaaggtcgcccgacgcccgggctttgcccgggcggcctcagtgagcgagcgagcgcgccagctggcgtaatagcgaagaggcccgcaccgatcgcccttcccaacagttgcgcagcctgaatggcgaatggcgattccgttgcaatggctggcggtaatattgttctggatattaccagcaaggccgatagtttgagttcttctactcaggcaagtgatgttattactaatcaaagaagtattgcgacaacggttaatttgcgtgatggacagactcttttactcggtggcctcactgattataaaaacacttctcaggattctggcgtaccgttcctgtctaaaatccctttaatcggcctcctgtttagctcccgctctgattctaacgaggaaagcacgttatacgtgctcgtcaaagcaaccatagtacgcgccctgtagcggcgcattaagcgcggcgggtgtggtggttacgcgcagcgtgaccgctacacttgccagcgccctagcgcccgctcctttcgctttcttcccttcctttctcgccacgttcgccggctttccccgtcaagctctaaatcgggggctccctttagggttccgatttagtgctttacggcacctcgaccccaaaaaacttgattagggtgatggttcacgtagtgggccatcgccctgatagacggtttttcgccctttgacgttggagtccacgttctttaatagtggactcttgttccaaactggaacaacactcaaccctatctcggtctattcttttgatttataagggattttgccgatttcggcctattggttaaaaaatgagctgatttaacaaaaatttaacgcgaattttaacaaaatattaacgtttacaatttaaatatttgcttatacaatcttcctgtttttggggcttttctgattatcaaccggggtacatatgattgacatgctagttttacgattaccgttcatcgattctcttgtttgctccagactctcaggcaatgacctgatagcctttgtagagacctctcaaaaatagctaccctctccggcatgaatttatcagctagaacggttgaatatcatattgatggtgatttgactgtctccggcctttctcacccgtttgaatctttacctacacattactcaggcattgcatttaaaatatatgagggttctaaaaatttttatccttgcgttgaaataaaggcttctcccgcaaaagtattacagggtcataatgtttttggtacaaccgatttagctttatgctctgaggctttattgcttaattttgctaattctttgccttgcctgtatgatttattggatgttggaatcgcctgatgcggtattttctccttacgcatctgtgcggtatttcacaccgcatatggtgcactctcagtacaatctgctctgatgccgcatagttaagccagccccgacacccgccaacacccgctgacgcgccctgacgggcttgtctgctcccggcatccgcttacagacaagctgtgaccgtctccgggagctgcatgtgtcagaggttttcaccgtcatcaccgaaacgcgcgagacgaaagggcctcgtgatacgcctatttttataggttaatgtcatgataataatggtttcttagacgtcaggtggcacttttcggggaaatgtgcgcggaacccctatttgtttatttttctaaatacattcaaatatgtatccgctcatgagacaataaccctgataaatgcttcaataatattgaaaaaggaagagtatgagtattcaacatttccgtgtcgcccttattcccttttttgcggcattttgccttcctgtttttgctcacccagaaacgctggtgaaagtaaaagatgctgaagatcagttgggtgcacgagtgggttacatcgaactggatctcaacagcggtaagatccttgagagttttcgccccgaagaacgttttccaatgatgagcacttttaaagttctgctatgtggcgcggtattatcccgtattgacgccgggcaagagcaactcggtcgccgcatacactattctcagaatgacttggttgagtactcaccagtcacagaaaagcatcttacggatggcatgacagtaagagaattatgcagtgctgccataaccatgagtgataacactgcggccaacttacttctgacaacgatcggaggaccgaaggagctaaccgcttttttgcacaacatgggggatcatgtaactcgccttgatcgttgggaaccggagctgaatgaagccataccaaacgacgagcgtgacaccacgatgcctgtagcaatggcaacaacgttgcgcaaactattaactggcgaactacttactctagcttcccggcaacaattaatagactggatggaggcggataaagttgcaggaccacttctgcgctcggcccttccggctggctggtttattgctgataaatctggagccggtgagcgtgggtctcgcggtatcattgcagcactggggccagatggtaagccctcccgtatcgtagttatctacacgacggggagtcaggcaactatggatgaacgaaatagacagatcgctgagataggtgcctcactgattaagcattggtaactgtcagaccaagtttactcatatatactttagattgatttaaaacttcatttttaatttaaaaggatctaggtgaagatcctttttgataatctcatgaccaaaatcccttaacgtgagttttcgttccactgagcgtcagaccccgtagaaaagatcaaaggatcttcttgagatcctttttttctgcgcgtaatctgctgcttgcaaacaaaaaaaccaccgctaccagcggtggtttgtttgccggatcaagagctaccaactctttttccgaaggtaactggcttcagcagagcgcagataccaaatactgtccttctagtgtagccgtagttaggccaccacttcaagaactctgtagcaccgcctacatacctcgctctgctaatcctgttaccagtggctgctgccagtggcgataagtcgtgtcttaccgggttggactcaagacgatagttaccggataaggcgcagcggtcgggctgaacggggggttcgtgcacacagcccagcttggagcgaacgacctacaccgaactgagatacctacagcgtgagctatgagaaagcgccacgcttcccgaagggagaaaggcggacaggtatccggtaagcggcagggtcggaacaggagagcgcacgagggagcttccagggggaaacgcctggtatctttatagtcctgtcgggtttcgccacctctgacttgagcgtcgatttttgtgatgctcgtcaggggggcggagcctatggaaaaacgccagcaacgcggcctttttacggttcctggccttttgctggccttttgctcacatgttctttcctgcgttatcccctgattctgtggataaccgtattaccgcctttgagtgagctgataccgctcgccgcagccgaacgaccgagcgcagcgagtcagtgagcgaggaagcggaagagcgcccaatacgcaaaccgcctctccccgcgcgttggccgattcattaatg

SEQ ID NO: 49 - DNA, 1325 bp, Homo sapiens
agtccagggctctgtcctgcacctggggaatggtgaccggcatctctgtcctctagctctggaagcaccccagcccctctagtctgccctcacccctgaccctgaccctccaccctgaccccgtcctaacccctgacctttgtgcccttccagagagaagggcagaagtgcccacagcccaccccagcccctcacccaggccagccggccagttccaaaccctggtggttggtgtcgtgggcggcctgctgggcagcctggtgctgctagtctgggtcctggccgtcatctgctcccgggccgcacgaggtaacgtcatcccagcccctcggcctgccctgccctaaccctgctggcggccctcactcccgcctccccttcctccacccttccctcaccccaccccacctccccccatctccccgccaggctaagtccctgatgaaggcccctggactaagaccccccacctaggagcacggctcagggtcggcctggtgaccccaagtgtgtttctctgcagggacaataggagccaggcgcaccggccagcccctggtgagtctcactcttttcctgcatgatccactgtgccttccttcctgggtgggcagaggtggaaggacaggctgggaccacacggcctgcaggactcacattctattatagccaggaccccacctccccagcccccaggcagcaacctcaatccctaaagccatgatctggggccccagcccacctgcggtctccgggggtgcccggcccatgtgtgtgcctgcctgcggtctccaggggtgcctggcccacgcgtgtgcccgcctgcggtctctgggggtgcccggcccacatatgtgcctgcctgcggtctccaggtgtgcccggcccatgcgtgtgcccacctgcgagggcgtggggtgggcttggtcatttcttatcttacattggagacaggagagcttgaaaagtcacattttggaatcctaaatctgcaagaatgccagggacatttcagagggggacattgagccagagaggaggggtggtgtccccagatcacacagagggcagtggtgggacagctcagggtaagcagctcgtagtggggggcccaggttcggtgccggtactgcagccaggctgtggagccgcgggcctccttcctgcggtgggccgtggggctgactccctctccctttctcctcaaagaaggaggacccctcagccgtgcctgtgttctctgtggactatggggagctggatttccagtggcgagagaagaccccggagccccccgtgccctgtgtccctgagcagacggagta

SEQ ID NO: 50 - DNA, 1072 bp, Homo sapiens
ccaccattgtctttcctagcggaatgggcacctcatcccccgcccgcaggggctcagccgacggccctcggagtgcccagccactgaggcctgaggatggacactgctcttggcccctctgaccggcttccttggccaccagtgttctgcagaccctccaccatgagcccgggtcagcgcatttcctcaggagaagcaggcagggtgcaggccattgcaggccgtccaggggctgagctgcctgggggcgaccggggctccagcctgcacctgcaccaggcacagccccaccacaggactcatgtctcaatgcccacagtgagcccaggcagcaggtgtcaccgtcccctacagggagggccagatgcagtcactgcttcaggtcctgccagcacagagctgcctgcgtccagctccctgaatctctgctgctgctgctgctgctgctgctgctgcctgcggcccggggctgaaggcgccgtggccctgcctgacgccccggagcctcctgcctgaacttgggggctggttggagatggccttggagcagccaaggtgcccctggcagtggcatcccgaaacgccctggacgcagggcccaagactgggcacaggagtgggaggtacatggggctggggactccccaggagttatctgctccctgcaggcctagagaagtttcagggaaggtcagaagagctcctggctgtggtgggcagggcaggaaacccctccacctttacacatgcccaggcagcacctcaggccctttgtggggcagggaagctgaggcagtaagcgggcaggcagagctggaggcctttcaggcccagccagcactctggcctcctgccgccgcattccaccccagcccctcacaccactcgggagagggacatcctacggtcccaaggtcaggagggcagggctggggttgactcaggcccctcccagctgtggccacctgggtgttgggagggcagaagtgcaggcacctagggccccccatgtgcccaccctgggagctctccttggaacccattcctgaaattatttaaaggggttggccgg

SEQ ID NO: 51 - DNA, 7880 bp, Artificial Sequence
  Synthesized rAAV PD-1 Exon5_MND-PD-1-CD28 Switch Receptor construct
cagctgcgcgctcgctcgctcactgaggccgcccgggcaaagcccgggcgtcgggcgacctttggtcgcccggcctcagtgagcgagcgagcgcgcagagagggagtggccaactccatcactaggggttccttgtagttaatgattaacccgccatgctacttatctacgtagaattcagtccagggctctgtcctgcacctggggaatggtgaccggcatctctgtcctctagctctggaagcaccccagcccctctagtctgccctcacccctgaccctgaccctccaccctgaccccgtcctaacccctgacctttgtgcccttccagagagaagggcagaagtgcccacagcccaccccagcccctcacccaggccagccggccagttccaaaccctggtggttggtgtcgtgggcggcctgctgggcagcctggtgctgctagtctgggtcctggccgtcatctgctcccgggccgcacgaggtaacgtcatcccagcccctcggcctgccctgccctaaccctgctggcggccctcactcccgcctccccttcctccacccttccctcaccccaccccacctccccccatctccccgccaggctaagtccctgatgaaggcccctggactaagaccccccacctaggagcacggctcagggtcggcctggtgaccccaagtgtgtttctctgcagggacaataggagccaggcgcaccggccagcccctggtgagtctcactcttttcctgcatgatccactgtgccttccttcctgggtgggcagaggtggaaggacaggctgggaccacacggcctgcaggactcacattctattatagccaggaccccacctccccagcccccaggcagcaacctcaatccctaaagccatgatctggggccccagcccacctgcggtctccgggggtgcccggcccatgtgtgtgcctgcctgcggtctccaggggtgcctggcccacgcgtgtgcccgcctgcggtctctgggggtgcccggcccacatatgtgcctgcctgcggtctccaggtgtgcccggcccatgcgtgtgcccacctgcgagggcgtggggtgggcttggtcatttcttatcttacattggagacaggagagcttgaaaagtcacattttggaatcctaaatctgcaagaatgccagggacatttcagagggggacattgagccagagaggaggggtggtgtccccagatcacacagagggcagtggtgggacagctcagggtaagcagctcatagtggggggcccaggttcggtgccggtactgcagccaggctgtggagccgcgggcctccttcctgcggtgggccgtggggctgactccctctccctttctcctcaaagaaggaggacccctcagccgtgcctgtgttctctgtggactatggggagctggatttccagtggcgagagaagaccccggagccccccgtgccctgtgtccctgagcagacggagtaatgcatgaacagagaaacaggagaatatgggccaaacaggatatctgtggtaagcagttcctgccccggctcagggccaagaacagttggaacagcagaatatgggccaaacaggatatctgtggtaagcagttcctgccccggctcagggccaagaacagatggtccccagatgcggtcccgccctcagcagtttctagagaaccatcagatgtttccagggtgccccaaggacctgaaatgaccctgtgccttatttgaactaaccaatcagttcgcttctcgcttctgttcgcgcgcttctgctccccgagctctatataagcagagctcgtttagtgaaccgtcagatcgcctggagacgccatccacgctgttttgacttccatagaaggatctcgaggccaccatgcagatcccgcaagcgccctggccagtcgtctgggcggtgctacaactgggctggcggccaggatggttcttagactccccagacaggccctggaacccccccaccttctccccagccctgctcgtggtgaccgaaggggacaacgccaccttcacctgcagcttctccaacacatcggagagcttcgtgctaaactggtaccgcatgagccccagcaaccagacggacaagctggccgccttccccgaggaccgcagccagcccggccaggactgccgcttccgtgtcacacaactgcccaacgggcgtgacttccacatgagcgtggtcagggcccggcgcaatgacagcggcacctacctctgtggggccatctccctggcccccaaggcgcagatcaaagagagcctgcgggcagagctcagggtgacagagagaagggcagaagtgcccacagcccaccccagcccctcacccaggccagccggccagttccaaaccctggtggttggtgtcgtgggcggcctgctgggcagcctggtgctgctagtctgggtcctggccgtcatcaggagtaagaggagcaggctcctgcacagtgactacatgaacatgactccccgccgccccgggcccacccgcaagcattaccagccctatgccccaccacgcgacttcgcagcctatcgctccggtgagggcagaggaagtcttctaacatgcggtgacgtggaggagaatccgggccctgtgagcaagggcgaggaggataactccgccatcatcaaggagttcctgcgcttcaaggtgcacatggagggctccgtgaacggccacgagttcgagatcgagggcgagggcgagggccgcccctacgagggcacccagaccgccaagctgaaggtgaccaagggtggccccctgcccttcgcctgggacatcctgtcccctcagttcatgtacggctccaaggcctacgtgaagcaccccgccgacatccccgactacttgaagctgtccttccccgagggcttcaagtgggagcgcgtgatgaacttcgaggacggcggcgtggtgaccgtgacccaggactcctctctgcaggacggcgagttcatctacaaggtgaagctgcgcggcaccaacttcccctccgacggccccgtaatgcagaagaagaccatgggctgggaggcctcctccgagcggatgtaccccgaggacggcgccctgaagggcgagatcaagcagaggctgaagctgaaggacggcggccactacgacgctgaggtcaagaccacctacaaggccaagaagcccgtgcagctgcccggcgcctacaacgtcaacatcaagttggacatcacctcccacaacgaggactacaccatcgtggaacagtacgaacgcgccgagggccgccactccaccggcggcatggacgagctgtacaagtgatgaaagctttgctttatttgtgaaatttgtgatgctattgctttatttgtaaccattataagctgcaataaacaagtttaacaacaacaattgcattcattttatgtttcaggttcagggggaggtgtgggaggttttttaaagtcgacgtggccctgcctgacgccccggagcctcctgcctgaacttgggggctggttggagatggccttggagcagccaaggtgcccctggcagtggcatcccgaaacgccctggacgcagggcccaagactgggcacaggagtgggaggtacatggggctggggactccccaggagttatctgctccctgcaggcctagagaagtttcagggaaggtcagaagagctcctggctgtggtgggcagggcaggaaacccctccacctttacacatgcccaggcagcacctcaggccctttgtggggcagggaagctgaggcagtaagcgggcaggcagagctggaggcctttcaggcccagccagcactctggcctcctgccgccgcattccaccccagcccctcacaccactcgggagagggacatcctacggtcccaaggtcaggagggcagggctggggttgactcaggcccctcccagctgtggccacctgggtgttgggagggcagaagtgcaggcacctagggccccccatgtgcccaccctgggagctctccttggaacccattcctgaaattatttaaaggggttggccggactagttacgtagataagtagcatggcgggttaatcattaactacaaggaacccctagtgatggagttggccactccctctctgcgcgctcgctcgctcactgaggccgggcgaccaaaggtcgcccgacgcccgggctttgcccgggcggcctcagtgagcgagcgagcgcgccagctggcgtaatagcgaagaggcccgcaccgatcgcccttcccaacagttgcgcagcctgaatggcgaatggcgattccgttgcaatggctggcggtaatattgttctggatattaccagcaaggccgatagtttgagttcttctactcaggcaagtgatgttattactaatcaaagaagtattgcgacaacggttaatttgcgtgatggacagactcttttactcggtggcctcactgattataaaaacacttctcaggattctggcgtaccgttcctgtctaaaatccctttaatcggcctcctgtttagctcccgctctgattctaacgaggaaagcacgttatacgtgctcgtcaaagcaaccatagtacgcgccctgtagcggcgcattaagcgcggcgggtgtggtggttacgcgcagcgtgaccgctacacttgccagcgccctagcgcccgctcctttcgctttcttcccttcctttctcgccacgttcgccggctttccccgtcaagctctaaatcgggggctccctttagggttccgatttagtgctttacggcacctcgaccccaaaaaacttgattagggtgatggttcacgtagtgggccatcgccctgatagacggtttttcgccctttgacgttggagtccacgttctttaatagtggactcttgttccaaactggaacaacactcaaccctatctcggtctattcttttgatttataagggattttgccgatttcggcctattggttaaaaaatgagctgatttaacaaaaatttaacgcgaattttaacaaaatattaacgtttacaatttaaatatttgcttatacaatcttcctgtttttggggcttttctgattatcaaccggggtacatatgattgacatgctagttttacgattaccgttcatcgattctcttgtttgctccagactctcaggcaatgacctgatagcctttgtagagacctctcaaaaatagctaccctctccggcatgaatttatcagctagaacggttgaatatcatattgatggtgatttgactgtctccggcctttctcacccgtttgaatctttacctacacattactcaggcattgcatttaaaatatatgagggttctaaaaatttttatccttgcgttgaaataaaggcttctcccgcaaaagtattacagggtcataatgtttttggtacaaccgatttagctttatgctctgaggctttattgcttaattttgctaattctttgccttgcctgtatgatttattggatgttggaatcgcctgatgcggtattttctccttacgcatctgtgcggtatttcacaccgcatatggtgcactctcagtacaatctgctctgatgccgcatagttaagccagccccgacacccgccaacacccgctgacgcgccctgacgggcttgtctgctcccggcatccgcttacagacaagctgtgaccgtctccgggagctgcatgtgtcagaggttttcaccgtcatcaccgaaacgcgcgagacgaaagggcctcgtgatacgcctatttttataggttaatgtcatgataataatggtttcttagacgtcaggtggcacttttcggggaaatgtgcgcggaacccctatttgtttatttttctaaatacattcaaatatgtatccgctcatgagacaataaccctgataaatgcttcaataatattgaaaaaggaagagtatgagtattcaacatttccgtgtcgcccttattcccttttttgcggcattttgccttcctgtttttgctcacccagaaacgctggtgaaagtaaaagatgctgaagatcagttgggtgcacgagtgggttacatcgaactggatctcaacagcggtaagatccttgagagttttcgccccgaagaacgttttccaatgatgagcacttttaaagttctgctatgtggcgcggtattatcccgtattgacgccgggcaagagcaactcggtcgccgcatacactattctcagaatgacttggttgagtactcaccagtcacagaaaagcatcttacggatggcatgacagtaagagaattatgcagtgctgccataaccatgagtgataacactgcggccaacttacttctgacaacgatcggaggaccgaaggagctaaccgcttttttgcacaacatgggggatcatgtaactcgccttgatcgttgggaaccggagctgaatgaagccataccaaacgacgagcgtgacaccacgatgcctgtagcaatggcaacaacgttgcgcaaactattaactggcgaactacttactctagcttcccggcaacaattaatagactggatggaggcggataaagttgcaggaccacttctgcgctcggcccttccggctggctggtttattgctgataaatctggagccggtgagcgtgggtctcgcggtatcattgcagcactggggccagatggtaagccctcccgtatcgtagttatctacacgacggggagtcaggcaactatggatgaacgaaatagacagatcgctgagataggtgcctcactgattaagcattggtaactgtcagaccaagtttactcatatatactttagattgatttaaaacttcatttttaatttaaaaggatctaggtgaagatcctttttgataatctcatgaccaaaatcccttaacgtgagttttcgttccactgagcgtcagaccccgtagaaaagatcaaaggatcttcttgagatcctttttttctgcgcgtaatctgctgcttgcaaacaaaaaaaccaccgctaccagcggtggtttgtttgccggatcaagagctaccaactctttttccgaaggtaactggcttcagcagagcgcagataccaaatactgtccttctagtgtagccgtagttaggccaccacttcaagaactctgtagcaccgcctacatacctcgctctgctaatcctgttaccagtggctgctgccagtggcgataagtcgtgtcttaccgggttggactcaagacgatagttaccggataaggcgcagcggtcgggctgaacggggggttcgtgcacacagcccagcttggagcgaacgacctacaccgaactgagatacctacagcgtgagctatgagaaagcgccacgcttcccgaagggagaaaggcggacaggtatccggtaagcggcagggtcggaacaggagagcgcacgagggagcttccagggggaaacgcctggtatctttatagtcctgtcgggtttcgccacctctgacttgagcgtcgatttttgtgatgctcgtcaggggggcggagcctatggaaaaacgccagcaacgcggcctttttacggttcctggccttttgctggccttttgctcacatgttctttcctgcgttatcccctgattctgtggataaccgtattaccgcctttgagtgagctgataccgctcgccgcagccgaacgaccgagcgcagcgagtcagtgagcgaggaagcggaagagcgcccaatacgcaaaccgcctctccccgcgcgttggccgattcattaatg

SEQ ID NO: 52 - DNA, 7593 bp, Artificial Sequence
  Synthesized rAAV PD-1 Exon5_MND-BFP_distal 5'-Homology Arm construct
cagctgcgcgctcgctcgctcactgaggccgcccgggcaaagcccgggcgtcgggcgacctttggtcgcccggcctcagtgagcgagcgagcgcgcagagagggagtggccaactccatcactaggggttccttgtagttaatgattaacccgccatgctacttatctacgtagaattcggccccactgcccactgcccagggcagcaatgcccataccacgtggtcccagctccgagcttgtcctgaaaagggggcaaagactggaccctgagcctgccaaggggccacactcctcccagggctggggtctccatgggcagccccccacccacccagaccagttacactcccctgtgccagagcagtgcagacaggaccaggccaggatgcccaagggtcaggggctggggatgggtagcccccaaacagccctttctgggggactggcctcaacggggaagggggtgaaggctcttagtaggaaatcagggagacccaagtcagagccaggcgctgtgcagaagctgcagcctcacgtagaaggaagagcctctgcagtggaggccagtgcccatccccgggtggcagaggccccagcagagacttctcaatgacattccagctggggtggcccttccagagcccttgctgcccgagggatgtgagcaggtggccggggaggctttgtggggccacccagccccttcctcacctctctccatctctcagactccccagacaggccctggaacccccccaccttctccccagccctgctcgtggtgaccgaaggggacaacgccaccttcacctgcagcttctccaacacatcggagagcttcgtgctaaactggtaccgcatgagccccagcaaccagacggacaagctggccgccttccccgaggaccgcagccagcccggccaggactgccgcttccgtgtcacacaactgcccaacgggcgtgacttccacatgagcgtggtcagggcccggcgcaatgacagcggcacctacctctgtggggccatctccctggcccccaaggcgcagatcaaagagagcctgcgggcagagctcagggtgacaggtgcggcctcggaggccccggggcaggggtgagctgagccggtcctggggtgggtgtcccctcctgcacaggatcaggagctccagggtcgtagggcagggaccccccagctccagtccagggctctgtcctgcacctggggaatggtgaccggcatctctgtcctctagctctggaagcaccccagcccctctagtctgccctcacccctgaccctgaccctccaccctgaccccgtcctaacccctgacctttgtgcccttccagagagaagggcagaagtgcccacagcccaccccagcccctcacccaggccagccggccagttccaaaccctggtggttggtgtcgtgggcggcctgctgggcagcctggtgctgctagtctgggtcctggccgtcatctatgcatgaacagagaaacaggagaatatgggccaaacaggatatctgtggtaagcagttcctgccccggctcagggccaagaacagttggaacagcagaatatgggccaaacaggatatctgtggtaagcagttcctgccccggctcagggccaagaacagatggtccccagatgcggtcccgccctcagcagtttctagagaaccatcagatgtttccagggtgccccaaggacctgaaatgaccctgtgccttatttgaactaaccaatcagttcgcttctcgcttctgttcgcgcgcttctgctccccgagctctatataagcagagctcgtttagtgaaccgtcagatcgcctggagacgccatccacgctgttttgacttccatagaaggatctcgaggccaccatggctagcgagctgattaaggagaacatgcacatgaagctgtacatggagggcaccgtggacaaccatcacttcaagtgcacatccgagggcgaaggcaagccctacgagggcacccagaccatgagaatcaaggtggtcgagggcggccctctccccttcgccttcgacatcctggctactagcttcctctacggcagcaagaccttcatcaaccacacccagggcatccccgacttcttcaagcagtccttccctgagggcttcacatgggagagagtcaccacatacgaggacgggggcgtgctgaccgctacccaggacaccagcctccaggacggctgcctcatctacaacgtcaagatcagaggggtgaacttcacatccaacggccctgtgatgcagaagaaaacactcggctgggaggccttcaccgagacgctgtaccccgctgacggcggcctggaaggcagaaacgacatggccctgaagctcgtgggcgggagccatctgatcgcaaacatcaagaccacatatagatccaagaaacccgctaagaacctcaagatgcctggcgtctactatgtggactacagactggaaagaatcaaggaggccaacaacgagacctacgtcgagcagcacgaggtggcagtggccagatactgcgacctccctagcaaactggggcacaagctaaattgaaagctttgctttatttgtgaaatttgtgatgctattgctttatttgtaaccattataagctgcaataaacaagtttaacaacaacaattgcattcattttatgtttcaggttcagggggaggtgtgggaggttttttaaagtcgacccaccattgtctttcctagcggaatgggcacctcatcccccgcccgcaggggctcagctgacggccctcggagtgcccagccactgaggcctgaggatggacactgctcttggcccctctgaccggcttccttggccaccagtgttctgcagaccctccaccatgagcccgggtcagcgcatttcctcaggagaagcaggcagggtgcaggccattgcaggccgtccaggggctgagctgcctgggggcgaccggggctccagcctgcacctgcaccaggcacagccccaccacaggactcatgtctcaatgcccacagtgagcccaggcagcaggtgtcaccgtcccctacagggagggccagatgcagtcactgcttcaggtcctgccagcacagagctgcctgcgtccagctccctgaatctctgctgctgctgctgctgctgctgctgctgcctgcggcccggggctgaaggcgccgtggccctgcctgacgccccggagcctcctgcctgaacttgggggctggttggagatggccttggagcagccaaggtgcccctggcagtggcatcccgaaacgccctggacgcagggcccaagactgggcacaggagtgggaggtacatggggctggggactccccaggagttatctgctccctgcaggcctagagaagtttcagggaaggtcagaagagctcctggctgtggtgggcagggcaggaaacccctccacctttacacatgcccaggcagcacctcaggccctttgtggggcagggaagctgaggcagtaagcgggcaggcagagctggaggcctttcaggcccagccagcactctggcctcctgccgccgcattccaccccagcccctcacaccactcgggagagggacatcctacggtcccaaggtcaggagggcagggctggggttgactcaggcccctcccagctgtggccacctgggtgttgggagggcagaagtgcaggcacctagggccccccatgtgcccaccctgggagctctccttggaacccattcctgaaattatttaaaggggttggccggactagttacgtagataagtagcatggcgggttaatcattaactacaaggaacccctagtgatggagttggccactccctctctgcgcgctcgctcgctcactgaggccgggcgaccaaaggtcgcccgacgcccgggctttgcccgggcggcctcagtgagcgagcgagcgcgccagctggcgtaatagcgaagaggcccgcaccgatcgcccttcccaacagttgcgcagcctgaatggcgaatggcgattccgttgcaatggctggcggtaatattgttctggatattaccagcaaggccgatagtttgagttcttctactcaggcaagtgatgttattactaatcaaagaagtattgcgacaacggttaatttgcgtgatggacagactcttttactcggtggcctcactgattataaaaacacttctcaggattctggcgtaccgttcctgtctaaaatccctttaatcggcctcctgtttagctcccgctctgattctaacgaggaaagcacgttatacgtgctcgtcaaagcaaccatagtacgcgccctgtagcggcgcattaagcgcggcgggtgtggtggttacgcgcagcgtgaccgctacacttgccagcgccctagcgcccgctcctttcgctttcttcccttcctttctcgccacgttcgccggctttccccgtcaagctctaaatcgggggctccctttagggttccgatttagtgctttacggcacctcgaccccaaaaaacttgattagggtgatggttcacgtagtgggccatcgccctgatagacggtttttcgccctttgacgttggagtccacgttctttaatagtggactcttgttccaaactggaacaacactcaaccctatctcggtctattcttttgatttataagggattttgccgatttcggcctattggttaaaaaatgagctgatttaacaaaaatttaacgcgaattttaacaaaatattaacgtttacaatttaaatatttgcttatacaatcttcctgtttttggggcttttctgattatcaaccggggtacatatgattgacatgctagttttacgattaccgttcatcgattctcttgtttgctccagactctcaggcaatgacctgatagcctttgtagagacctctcaaaaatagctaccctctccggcatgaatttatcagctagaacggttgaatatcatattgatggtgatttgactgtctccggcctttctcacccgtttgaatctttacctacacattactcaggcattgcatttaaaatatatgagggttctaaaaatttttatccttgcgttgaaataaaggcttctcccgcaaaagtattacagggtcataatgtttttggtacaaccgatttagctttatgctctgaggctttattgcttaattttgctaattctttgccttgcctgtatgatttattggatgttggaatcgcctgatgcggtattttctccttacgcatctgtgcggtatttcacaccgcatatggtgcactctcagtacaatctgctctgatgccgcatagttaagccagccccgacacccgccaacacccgctgacgcgccctgacgggcttgtctgctcccggcatccgcttacagacaagctgtgaccgtctccgggagctgcatgtgtcagaggttttcaccgtcatcaccgaaacgcgcgagacgaaagggcctcgtgatacgcctatttttataggttaatgtcatgataataatggtttcttagacgtcaggtggcacttttcggggaaatgtgcgcggaacccctatttgtttatttttctaaatacattcaaatatgtatccgctcatgagacaataaccctgataaatgcttcaataatattgaaaaaggaagagtatgagtattcaacatttccgtgtcgcccttattcccttttttgcggcattttgccttcctgtttttgctcacccagaaacgctggtgaaagtaaaagatgctgaagatcagttgggtgcacgagtgggttacatcgaactggatctcaacagcggtaagatccttgagagttttcgccccgaagaacgttttccaatgatgagcacttttaaagttctgctatgtggcgcggtattatcccgtattgacgccgggcaagagcaactcggtcgccgcatacactattctcagaatgacttggttgagtactcaccagtcacagaaaagcatcttacggatggcatgacagtaagagaattatgcagtgctgccataaccatgagtgataacactgcggccaacttacttctgacaacgatcggaggaccgaaggagctaaccgcttttttgcacaacatgggggatcatgtaactcgccttgatcgttgggaaccggagctgaatgaagccataccaaacgacgagcgtgacaccacgatgcctgtagcaatggcaacaacgttgcgcaaactattaactggcgaactacttactctagcttcccggcaacaattaatagactggatggaggcggataaagttgcaggaccacttctgcgctcggcccttccggctggctggtttattgctgataaatctggagccggtgagcgtgggtctcgcggtatcattgcagcactggggccagatggtaagccctcccgtatcgtagttatctacacgacggggagtcaggcaactatggatgaacgaaatagacagatcgctgagataggtgcctcactgattaagcattggtaactgtcagaccaagtttactcatatatactttagattgatttaaaacttcatttttaatttaaaaggatctaggtgaagatcctttttgataatctcatgaccaaaatcccttaacgtgagttttcgttccactgagcgtcagaccccgtagaaaagatcaaaggatcttcttgagatcctttttttctgcgcgtaatctgctgcttgcaaacaaaaaaaccaccgctaccagcggtggtttgtttgccggatcaagagctaccaactctttttccgaaggtaactggcttcagcagagcgcagataccaaatactgtccttctagtgtagccgtagttaggccaccacttcaagaactctgtagcaccgcctacatacctcgctctgctaatcctgttaccagtggctgctgccagtggcgataagtcgtgtcttaccgggttggactcaagacgatagttaccggataaggcgcagcggtcgggctgaacggggggttcgtgcacacagcccagcttggagcgaacgacctacaccgaactgagatacctacagcgtgagctatgagaaagcgccacgcttcccgaagggagaaaggcggacaggtatccggtaagcggcagggtcggaacaggagagcgcacgagggagcttccagggggaaacgcctggtatctttatagtcctgtcgggtttcgccacctctgacttgagcgtcgatttttgtgatgctcgtcaggggggcggagcctatggaaaaacgccagcaacgcggcctttttacggttcctggccttttgctggccttttgctcacatgttctttcctgcgttatcccctgattctgtggataaccgtattaccgcctttgagtgagctgataccgctcgccgcagccgaacgaccgagcgcagcgagtcagtgagcgaggaagcggaagagcgcccaatacgcaaaccgcctctccccgcgcgttggccgattcattaatg

SEQ ID NO: 53 - DNA, 6718 bp, Artificial Sequence
  Synthesized rAAV PD-1 Exon1_MND-GFP construct
cagctgcgcgctcgctcgctcactgaggccgcccgggcaaagcccgggcgtcgggcgacctttggtcgcccggcctcagtgagcgagcgagcgcgcagagagggagtggccaactccatcactaggggttccttgtagttaatgattaacccgccatgctacttatctacgtaaggctgttgcaggcatcacacggtggaaagatctggaactgtggccatggtgtgaggccatccacaaggtggaagctttgagggggagccgattagccatggacagttgtcattcagtagggtcacctgtgccccagcgaagggggatgggccgggaaggcagaggccaggcacctgcccccagcaggggcagaggctgtgggcagccgggaggctcccagaggctccgacagaatgggagtggggttgagcccacccctcactgcagcccaggaacctgagcccagagggggccacccaccttccccaggcagggaggcccggcccccagggagatgggggggatgggggaggagaagggcctgcccccacccggcagcctcaggaggggcagctcgggcgggatatggaaagaggccacagcagtgagcagagacacagaggaggaaggggccctgagctggggagacccccacggggtagggcgtgggggccacgggcccacctcctccccatctcctctgtctccctgtctctgtctctctctccctcccccaccctctccccagtcctaccccctcctcacccctcctcccccagcactgcctctgtcactctcgcccacgtggatgtggaggaagagggggcgggagcaaggggcgggcaccctcccttcaacctgacctgggacagtttcccttccgctcacctccgcctgagcagtggagaaggcggcactctggtggggctgctccaacgcgtgaacagagaaacaggagaatatgggccaaacaggatatctgtggtaagcagttcctgccccggctcagggccaagaacagttggaacagcagaatatgggccaaacaggatatctgtggtaagcagttcctgccccggctcagggccaagaacagatggtccccagatgcggtcccgccctcagcagtttctagagaaccatcagatgtttccagggtgccccaaggacctgaaatgaccctgtgccttatttgaactaaccaatcagttcgcttctcgcttctgttcgcgcgcttctgctccccgagctctatataagcagagctcgtttagtgaaccgtcagatcgcctggagacgccatccacgctgttttgacttccatagaaggatctcgaggccaccatggtgagcaagggcgaggagctgttcaccggggtggtgcccatcctggtcgagctggacggcgacgtaaacggccacaagttcagcgtgtccggcgagggcgagggcgatgccacctacggcaagctgaccctgaagttcatctgcaccaccggcaagctgcccgtgccctggcccaccctcgtgaccaccctgacctacggcgtgcagtgcttcagccgctaccccgaccacatgaagcagcacgacttcttcaagtccgccatgcccgaaggctacgtccaggagcgcaccatcttcttcaaggacgacggcaactacaagacccgcgccgaggtgaagttcgagggcgacaccctggtgaaccgcatcgagctgaagggcatcgacttcaaggaggacggcaacatcctggggcacaagctggagtacaactacaacagccacaacgtctatatcatggccgacaagcagaagaacggcatcaaggtgaacttcaagatccgccacaacatcgaggacggcagcgtgcagctcgccgaccactaccagcagaacacccccatcggcgacggccccgtgctgctgcccgacaaccactacctgagcacccagtccgccctgagcaaagaccccaacgagaagcgcgatcacatggtcctgctggagttcgtgaccgccgccgggatcactctcggcatggacgagctgtacaagtaagcggccgcgctttatttgtgaaatttgtgatgctattgctttatttgtaaccattataagctgcaataaacaagttaacaacaacaattgcattcattttatgtttcaggttcagggggagatgtgggaggttttttaaagcctcaccggttctgggcggtgctacaactgggctggcggccaggatggttcttaggtaggtggggtcggcggtcaggtgtcccagagccaggggtctggagggaccttccaccctcagtccctggcaggtcggggggtgctgaggcgggcctggccctggcagcccaggggtcccggagcgaggggtctggagggacctttcactctcagtccctggcaggtcggggggtgctgtggcaggcccagccttggcccccagctctgccccttaccctgagctgtgtggctttgggcagctcgaactcctgggttcctctctgggccccaactcctcccctggcccaagtcccctctttgctcctgggcaggcaggacctctgtcccctctcagccggtccttggggctgcgtgtttctgtagaatgacgggtcaggctggccagaaccccaaaccttggccgtggggagtctgcgtggcggctctgccttgcccaggcatccttggtcctcactcgagttttcctaaggatgggatgagccccatgtgggactaaccttggctttacgacgtcaaagtttagatgagctggtgatatttttctcattatatccaaagtgtacctgttcgagtgaggacagttcttctgtctccaggatccctcctgggtggggattgtgcccgcctgggtctctgcccagattccagggctctccccgagccctgttcagaccatccgtgggggaggccttggcctcactcttacgtagataagtagcatggcgggttaatcattaactacaaggaacccctagtgatggagttggccactccctctctgcgcgctcgctcgctcactgaggccgggcgaccaaaggtcgcccgacgcccgggctttgcccgggcggcctcagtgagcgagcgagcgcgccagctggcgtaatagcgaagaggcccgcaccgatcgcccttcccaacagttgcgcagcctgaatggcgaatggcgattccgttgcaatggctggcggtaatattgttctggatattaccagcaaggccgatagtttgagttcttctactcaggcaagtgatgttattactaatcaaagaagtattgcgacaacggttaatttgcgtgatggacagactcttttactcggtggcctcactgattataaaaacacttctcaggattctggcgtaccgttcctgtctaaaatccctttaatcggcctcctgtttagctcccgctctgattctaacgaggaaagcacgttatacgtgctcgtcaaagcaaccatagtacgcgccctgtagcggcgcattaagcgcggcgggtgtggtggttacgcgcagcgtgaccgctacacttgccagcgccctagcgcccgctcctttcgctttcttcccttcctttctcgccacgttcgccggctttccccgtcaagctctaaatcgggggctccctttagggttccgatttagtgctttacggcacctcgaccccaaaaaacttgattagggtgatggttcacgtagtgggccatcgccctgatagacggtttttcgccctttgacgttggagtccacgttctttaatagtggactcttgttccaaactggaacaacactcaaccctatctcggtctattcttttgatttataagggattttgccgatttcggcctattggttaaaaaatgagctgatttaacaaaaatttaacgcgaattttaacaaaatattaacgtttacaatttaaatatttgcttatacaatcttcctgtttttggggcttttctgattatcaaccggggtacatatgattgacatgctagttttacgattaccgttcatcgattctcttgtttgctccagactctcaggcaatgacctgatagcctttgtagagacctctcaaaaatagctaccctctccggcatgaatttatcagctagaacggttgaatatcatattgatggtgatttgactgtctccggcctttctcacccgtttgaatctttacctacacattactcaggcattgcatttaaaatatatgagggttctaaaaatttttatccttgcgttgaaataaaggcttctcccgcaaaagtattacagggtcataatgtttttggtacaaccgatttagctttatgctctgaggctttattgcttaattttgctaattctttgccttgcctgtatgatttattggatgttggaatcgcctgatgcggtattttctccttacgcatctgtgcggtatttcacaccgcatatggtgcactctcagtacaatctgctctgatgccgcatagttaagccagccccgacacccgccaacacccgctgacgcgccctgacgggcttgtctgctcccggcatccgcttacagacaagctgtgaccgtctccgggagctgcatgtgtcagaggttttcaccgtcatcaccgaaacgcgcgagacgaaagggcctcgtgatacgcctatttttataggttaatgtcatgataataatggtttcttagacgtcaggtggcacttttcggggaaatgtgcgcggaacccctatttgtttatttttctaaatacattcaaatatgtatccgctcatgagacaataaccctgataaatgcttcaataatattgaaaaaggaagagtatgagtattcaacatttccgtgtcgcccttattcccttttttgcggcattttgccttcctgtttttgctcacccagaaacgctggtgaaagtaaaagatgctgaagatcagttgggtgcacgagtgggttacatcgaactggatctcaacagcggtaagatccttgagagttttcgccccgaagaacgttttccaatgatgagcacttttaaagttctgctatgtggcgcggtattatcccgtattgacgccgggcaagagcaactcggtcgccgcatacactattctcagaatgacttggttgagtactcaccagtcacagaaaagcatcttacggatggcatgacagtaagagaattatgcagtgctgccataaccatgagtgataacactgcggccaacttacttctgacaacgatcggaggaccgaaggagctaaccgcttttttgcacaacatgggggatcatgtaactcgccttgatcgttgggaaccggagctgaatgaagccataccaaacgacgagcgtgacaccacgatgcctgtagcaatggcaacaacgttgcgcaaactattaactggcgaactacttactctagcttcccggcaacaattaatagactggatggaggcggataaagttgcaggaccacttctgcgctcggcccttccggctggctggtttattgctgataaatctggagccggtgagcgtgggtctcgcggtatcattgcagcactggggccagatggtaagccctcccgtatcgtagttatctacacgacggggagtcaggcaactatggatgaacgaaatagacagatcgctgagataggtgcctcactgattaagcattggtaactgtcagaccaagtttactcatatatactttagattgatttaaaacttcatttttaatttaaaaggatctaggtgaagatcctttttgataatctcatgaccaaaatcccttaacgtgagttttcgttccactgagcgtcagaccccgtagaaaagatcaaaggatcttcttgagatcctttttttctgcgcgtaatctgctgcttgcaaacaaaaaaaccaccgctaccagcggtggtttgtttgccggatcaagagctaccaactctttttccgaaggtaactggcttcagcagagcgcagataccaaatactgtccttctagtgtagccgtagttaggccaccacttcaagaactctgtagcaccgcctacatacctcgctctgctaatcctgttaccagtggctgctgccagtggcgataagtcgtgtcttaccgggttggactcaagacgatagttaccggataaggcgcagcggtcgggctgaacggggggttcgtgcacacagcccagcttggagcgaacgacctacaccgaactgagatacctacagcgtgagctatgagaaagcgccacgcttcccgaagggagaaaggcggacaggtatccggtaagcggcagggtcggaacaggagagcgcacgagggagcttccagggggaaacgcctggtatctttatagtcctgtcgggtttcgccacctctgacttgagcgtcgatttttgtgatgctcgtcaggggggcggagcctatggaaaaacgccagcaacgcggcctttttacggttcctggccttttgctggccttttgctcacatgttctttcctgcgttatcccctgattctgtggataaccgtattaccgcctttgagtgagctgataccgctcgccgcagccgaacgaccgagcgcagcgagtcagtgagcgaggaagcggaagagcgcccaatacgcaaaccgcctctccccgcgcgttggccgattcattaatg

SEQ ID NO: 54 - DNA, 756 bp, Homo sapiens
aggctgttgcaggcatcacacggtggaaagatctggaactgtggccatggtgtgaggccatccacaaggtggaagctttgagggggagccgattagccatggacagttgtcattcagtagggtcacctgtgccccagcgaagggggatgggccgggaaggcagaggccaggcacctgcccccagcaggggcagaggctgtgggcagccgggaggctcccagaggctccgacagaatgggagtggggttgagcccacccctcactgcagcccaggaacctgagcccagagggggccacccaccttccccaggcagggaggcccggcccccagggagatgggggggatgggggaggagaagggcctgcccccacccggcagcctcaggaggggcagctcgggcgggatatggaaagaggccacagcagtgagcagagacacagaggaggaaggggccctgagctggggagacccccacggggtagggcgtgggggccacgggcccacctcctccccatctcctctgtctccctgtctctgtctctctctccctcccccaccctctccccagtcctaccccctcctcacccctcctcccccagcactgcctctgtcactctcgcccacgtggatgtggaggaagagggggcgggagcaaggggcgggcaccctcccttcaacctgacctgggacagtttcccttccgctcacctccgcctgagcagtggagaaggcggcactctggtggggctgctcca

SEQ ID NO: 55 - DNA, 750 bp, Homo sapiens
tctgggcggtgctacaactgggctggcggccaggatggttcttaggtaggtggggtcggcggtcaggtgtcccagagccaggggtctggagggaccttccaccctcagtccctggcaggtcggggggtgctgaggcgggcctggccctggcagcccaggggtcccggagcgaggggtctggagggacctttcactctcagtccctggcaggtcggggggtgctgtggcaggcccagccttggcccccagctctgccccttaccctgagctgtgtggctttgggcagctcgaactcctgggttcctctctgggccccaactcctcccctggcccaagtcccctctttgctcctgggcaggcaggacctctgtcccctctcagccggtccttggggctgcgtgtttctgtagaatgacgggtcaggctggccagaaccccaaaccttggccgtggggagtctgcgtggcggctctgccttgcccaggcatccttggtcctcactcgagttttcctaaggatgggatgagccccatgtgggactaaccttggctttacgacgtcaaagtttagatgagctggtgatatttttctcattatatccaaagtgtacctgttcgagtgaggacagttcttctgtctccaggatccctcctgggtggggattgtgcccgcctgggtctctgcccagattccagggctctccccgagccctgttcagaccatccgtgggggaggccttggcctcactct

SEQ ID NO: 56 - DNA, 7609 bp, Artificial Sequence
  Synthesized rAAV PD-1 Exon1_MND-CD19CAR construct
cagctgcgcgctcgctcgctcactgaggccgcccgggcaaagcccgggcgtcgggcgacctttggtcgcccggcctcagtgagcgagcgagcgcgcagagagggagtggccaactccatcactaggggttccttgtagttaatgattaacccgccatgctacttatctacgtaaggctgttgcaggcatcacacggtggaaagatctggaactgtggccatggtgtgaggccatccacaaggtggaagctttgagggggagccgattagccatggacagttgtcattcagtagggtcacctgtgccccagcgaagggggatgggccgggaaggcagaggccaggcacctgcccccagcaggggcagaggctgtgggcagccgggaggctcccagaggctccgacagaatgggagtggggttgagcccacccctcactgcagcccaggaacctgagcccagagggggccacccaccttccccaggcagggaggcccggcccccagggagatgggggggatgggggaggagaagggcctgcccccacccggcagcctcaggaggggcagctcgggcgggatatggaaagaggccacagcagtgagcagagacacagaggaggaaggggccctgagctggggagacccccacggggtagggcgtgggggccacgggcccacctcctccccatctcctctgtctccctgtctctgtctctctctccctcccccaccctctccccagtcctaccccctcctcacccctcctcccccagcactgcctctgtcactctcgcccacgtggatgtggaggaagagggggcgggagcaaggggcgggcaccctcccttcaacctgacctgggacagtttcccttccgctcacctccgcctgagcagtggagaaggcggcactctggtggggctgctccaacgcgtgatccatcgattagtccaatttgttaaagacaggatatcagtggtccaggctctagttttgactcaacaatatcaccagctgaagcctatagagtacgagccatagatagaataaaagattttatttagtctccagaaaaaggggggaatgaaagaccccacctgtaggtttggcaagctaggatcaaggttaggaacagagagacagcagaatatgggccaaacaggatatctgtggtaagcagttcctgccccggctcagggccaagaacagttggaacagcagaatatgggccaaacaggatatctgtggtaagcagttcctgccccggctcagggccaagaacagatggtccccagatgcggtcccgccctcagcagtttctagagaaccatcagatgtttccagggtgccccaaggacctgaaatgaccctgtgccttatttgaactaaccaatcagttcgcttctcgcttctgttcgcgcgcttctgctccccgagctcaataaaagagcccacaacccctcactcggcgcgacgcgtcatagccaccatggccttaccagtgaccgccttgctcctgccgctggccttgctgctccacgccgccaggccggacatccagatgacacagactacatcctccctgtctgcctctctgggagacagagtcaccatcagttgcagggcaagtcaggacattagtaaatatttaaattggtatcagcagaaaccagatggaactgttaaactcctgatctaccatacatcaagattacactcaggagtcccatcaaggttcagtggcagtgggtctggaacagattattctctcaccattagcaacctggagcaagaagatattgccacttacttttgccaacagggtaatacgcttccgtacacgttcggaggggggaccaagctggagatcacaggtggcggtggctccggcggtggtgggtctggtggcggcggaagcgaggtgaaactgcaggagtcaggacctggcctggtggcgccctcacagagcctgtccgtcacatgcactgtctcaggggtctcattacccgactatggtgtaagctggattcgccagcctccacgaaagggtctggagtggctgggagtaatatggggtagtgaaaccacatactataattcagctctcaaatccagactgaccatcatcaaggacaactccaagagccaagttttcttaaaaatgaacagtctgcaaactgatgacacagccatttactactgtgccaaacattattactacggtggtagctatgctatggactactggggtcaaggaacctcggtcaccgtctcctcaaccacgacgccagcgccgcgaccaccaacaccggcgcccaccatcgcgtcgcagcccctgtccctgcgcccagaggcgtgccggccagcggcggggggcgcagtgcacacgagggggctggacttcgcctgtgatatctacatctgggcgcccttggccgggacttgtggggtccttctcctgtcactggtgatcaccctttactgcaaacggggcagaaagaaactcctgtatatattcaaacaaccatttatgagaccagtacaaactactcaagaggaagatggctgtagctgccgatttccagaagaagaagaaggaggatgtgaactgagagtgaagttcagcaggagcgcagacgcccccgcgtaccagcagggccagaaccagctctataacgagctcaatctaggacgaagagaggagtacgatgttttggacaagagacgtggccgggaccctgagatggggggaaagccgagaaggaagaaccctcaggaaggcctgtacaatgaactgcagaaagataagatggcggaggcctacagtgagattgggatgaaaggcgagcgccggaggggcaaggggcacgatggcctttaccagggtctcagtacagccaccaaggacacctacgacgcccttcacatgcaggccctgccccctcgctaagcggccgcgctttatttgtgaaatttgtgatgctattgctttatttgtaaccattataagctgcaataaacaagttaacaacaacaattgcattcattttatgtttcaggttcagggggagatgtgggaggttttttaaagctcaccggttctgggcggtgctacaactgggctggcggccaggatggttcttaggtaggtggggtcggcggtcaggtgtcccagagccaggggtctggagggaccttccaccctcagtccctggcaggtcggggggtgctgaggcgggcctggccctggcagcccaggggtcccggagcgaggggtctggagggacctttcactctcagtccctggcaggtcggggggtgctgtggcaggcccagccttggcccccagctctgccccttaccctgagctgtgtggctttgggcagctcgaactcctgggttcctctctgggccccaactcctcccctggcccaagtcccctctttgctcctgggcaggcaggacctctgtcccctctcagccggtccttggggctgcgtgtttctgtagaatgacgggtcaggctggccagaaccccaaaccttggccgtggggagtctgcgtggcggctctgccttgcccaggcatccttggtcctcactcgagttttcctaaggatgggatgagccccatgtgggactaaccttggctttacgacgtcaaagtttagatgagctggtgatatttttctcattatatccaaagtgtacctgttcgagtgaggacagttcttctgtctccaggatccctcctgggtggggattgtgcccgcctgggtctctgcccagattccagggctctccccgagccctgttcagaccatccgtgggggaggccttggcctcactcttacgtagataagtagcatggcgggttaatcattaactacaaggaacccctagtgatggagttggccactccctctctgcgcgctcgctcgctcactgaggccgggcgaccaaaggtcgcccgacgcccgggctttgcccgggcggcctcagtgagcgagcgagcgcgccagctggcgtaatagcgaagaggcccgcaccgatcgcccttcccaacagttgcgcagcctgaatggcgaatggcgattccgttgcaatggctggcggtaatattgttctggatattaccagcaaggccgatagtttgagttcttctactcaggcaagtgatgttattactaatcaaagaagtattgcgacaacggttaatttgcgtgatggacagactcttttactcggtggcctcactgattataaaaacacttctcaggattctggcgtaccgttcctgtctaaaatccctttaatcggcctcctgtttagctcccgctctgattctaacgaggaaagcacgttatacgtgctcgtcaaagcaaccatagtacgcgccctgtagcggcgcattaagcgcggcgggtgtggtggttacgcgcagcgtgaccgctacacttgccagcgccctagcgcccgctcctttcgctttcttcccttcctttctcgccacgttcgccggctttccccgtcaagctctaaatcgggggctccctttagggttccgatttagtgctttacggcacctcgaccccaaaaaacttgattagggtgatggttcacgtagtgggccatcgccctgatagacggtttttcgccctttgacgttggagtccacgttctttaatagtggactcttgttccaaactggaacaacactcaaccctatctcggtctattcttttgatttataagggattttgccgatttcggcctattggttaaaaaatgagctgatttaacaaaaatttaacgcgaattttaacaaaatattaacgtttacaatttaaatatttgcttatacaatcttcctgtttttggggcttttctgattatcaaccggggtacatatgattgacatgctagttttacgattaccgttcatcgattctcttgtttgctccagactctcaggcaatgacctgatagcctttgtagagacctctcaaaaatagctaccctctccggcatgaatttatcagctagaacggttgaatatcatattgatggtgatttgactgtctccggcctttctcacccgtttgaatctttacctacacattactcaggcattgcatttaaaatatatgagggttctaaaaatttttatccttgcgttgaaataaaggcttctcccgcaaaagtattacagggtcataatgtttttggtacaaccgatttagctttatgctctgaggctttattgcttaattttgctaattctttgccttgcctgtatgatttattggatgttggaatcgcctgatgcggtattttctccttacgcatctgtgcggtatttcacaccgcatatggtgcactctcagtacaatctgctctgatgccgcatagttaagccagccccgacacccgccaacacccgctgacgcgccctgacgggcttgtctgctcccggcatccgcttacagacaagctgtgaccgtctccgggagctgcatgtgtcagaggttttcaccgtcatcaccgaaacgcgcgagacgaaagggcctcgtgatacgcctatttttataggttaatgtcatgataataatggtttcttagacgtcaggtggcacttttcggggaaatgtgcgcggaacccctatttgtttatttttctaaatacattcaaatatgtatccgctcatgagacaataaccctgataaatgcttcaataatattgaaaaaggaagagtatgagtattcaacatttccgtgtcgcccttattcccttttttgcggcattttgccttcctgtttttgctcacccagaaacgctggtgaaagtaaaagatgctgaagatcagttgggtgcacgagtgggttacatcgaactggatctcaacagcggtaagatccttgagagttttcgccccgaagaacgttttccaatgatgagcacttttaaagttctgctatgtggcgcggtattatcccgtattgacgccgggcaagagcaactcggtcgccgcatacactattctcagaatgacttggttgagtactcaccagtcacagaaaagcatcttacggatggcatgacagtaagagaattatgcagtgctgccataaccatgagtgataacactgcggccaacttacttctgacaacgatcggaggaccgaaggagctaaccgcttttttgcacaacatgggggatcatgtaactcgccttgatcgttgggaaccggagctgaatgaagccataccaaacgacgagcgtgacaccacgatgcctgtagcaatggcaacaacgttgcgcaaactattaactggcgaactacttactctagcttcccggcaacaattaatagactggatggaggcggataaagttgcaggaccacttctgcgctcggcccttccggctggctggtttattgctgataaatctggagccggtgagcgtgggtctcgcggtatcattgcagcactggggccagatggtaagccctcccgtatcgtagttatctacacgacggggagtcaggcaactatggatgaacgaaatagacagatcgctgagataggtgcctcactgattaagcattggtaactgtcagaccaagtttactcatatatactttagattgatttaaaacttcatttttaatttaaaaggatctaggtgaagatcctttttgataatctcatgaccaaaatcccttaacgtgagttttcgttccactgagcgtcagaccccgtagaaaagatcaaaggatcttcttgagatcctttttttctgcgcgtaatctgctgcttgcaaacaaaaaaaccaccgctaccagcggtggtttgtttgccggatcaagagctaccaactctttttccgaaggtaactggcttcagcagagcgcagataccaaatactgtccttctagtgtagccgtagttaggccaccacttcaagaactctgtagcaccgcctacatacctcgctctgctaatcctgttaccagtggctgctgccagtggcgataagtcgtgtcttaccgggttggactcaagacgatagttaccggataaggcgcagcggtcgggctgaacggggggttcgtgcacacagcccagcttggagcgaacgacctacaccgaactgagatacctacagcgtgagctatgagaaagcgccacgcttcccgaagggagaaaggcggacaggtatccggtaagcggcagggtcggaacaggagagcgcacgagggagcttccagggggaaacgcctggtatctttatagtcctgtcgggtttcgccacctctgacttgagcgtcgatttttgtgatgctcgtcaggggggcggagcctatggaaaaacgccagcaacgcggcctttttacggttcctggccttttgctggccttttgctcacatgttctttcctgcgttatcccctgattctgtggataaccgtattaccgcctttgagtgagctgataccgctcgccgcagccgaacgaccgagcgcagcgagtcagtgagcgaggaagcggaagagcgcccaatacgcaaaccgcctctccccgcgcgttggccgattcattaatg

SEQ ID NO: 57 - DNA, 7492 bp, Artificial Sequence
  Synthesized rAAV PD-1 Exon1_MND-BCMACAR construct
cagctgcgcgctcgctcgctcactgaggccgcccgggcaaagcccgggcgtcgggcgacctttggtcgcccggcctcagtgagcgagcgagcgcgcagagagggagtggccaactccatcactaggggttccttgtagttaatgattaacccgccatgctacttatctacgtaaggctgttgcaggcatcacacggtggaaagatctggaactgtggccatggtgtgaggccatccacaaggtggaagctttgagggggagccgattagccatggacagttgtcattcagtagggtcacctgtgccccagcgaagggggatgggccgggaaggcagaggccaggcacctgcccccagcaggggcagaggctgtgggcagccgggaggctcccagaggctccgacagaatgggagtggggttgagcccacccctcactgcagcccaggaacctgagcccagagggggccacccaccttccccaggcagggaggcccggcccccagggagatgggggggatgggggaggagaagggcctgcccccacccggcagcctcaggaggggcagctcgggcgggatatggaaagaggccacagcagtgagcagagacacagaggaggaaggggccctgagctggggagacccccacggggtagggcgtgggggccacgggcccacctcctccccatctcctctgtctccctgtctctgtctctctctccctcccccaccctctccccagtcctaccccctcctcacccctcctcccccagcactgcctctgtcactctcgcccacgtggatgtggaggaagagggggcgggagcaaggggcgggcaccctcccttcaacctgacctgggacagtttcccttccgctcacctccgcctgagcagtggagaaggcggcactctggtggggctgctccaacgcgtaatgaaagaccccacctgtaggtttggcaagctaggatcaaggttaggaacagagagacagcagaatatgggccaaacaggatatctgtggtaagcagttcctgccccggctcagggccaagaacagttggaacagcagaatatgggccaaacaggatatctgtggtaagcagttcctgccccggctcagggccaagaacagatggtccccagatgcggtcccgccctcagcagtttctagagaaccatcagatgtttccagggtgccccaaggacctgaaatgaccctgtgccttatttgaactaaccaatcagttcgcttctcgcttctgttcgcgcgcttctgctccccgagctcaataaaagagcccacaacccctcactcggcgcgattcacctgacgcgtctacgccaccatggcactccccgtcaccgcccttctcttgcccctcgccctgctgctgcatgctgccaggcccgacattgtgctcactcagtcacctcccagcctggccatgagcctgggaaaaagggccaccatctcctgtagagccagtgagtccgtcacaatcttggggagccatcttattcactggtatcagcagaagcccgggcagcctccaacccttcttattcagctcgcgtcaaacgtccagacgggtgtacctgccagattttctggtagcgggtcccgcactgattttacactgaccatagatccagtggaagaagacgatgtggccgtgtattattgtctgcagagcagaacgattcctcgcacatttggtgggggtactaagctggagattaagggaagcacgtccggctcagggaagccgggctccggcgagggaagcacgaaggggcaaattcagctggtccagagcggacctgagctgaaaaaacccggcgagactgttaagatcagttgtaaagcatctggctataccttcaccgactacagcataaattgggtgaaacgggcccctggaaagggcctcaaatggatgggttggatcaataccgaaactagggagcctgcttatgcatatgacttccgcgggagattcgccttttcactcgagacatctgcctctactgcttacctccaaataaacaacctcaagtatgaagatacagccacttacttttgcgccctcgactatagttacgccatggactactggggacagggaacctccgttaccgtcagttccgcggccgcaaccacaacacctgctccaaggccccccacacccgctccaactatagccagccaaccattgagcctcagacctgaagcttgcaggcccgcagcaggaggcgccgtccatacgcgaggcctggacttcgcgtgtgatatttatatttgggcccctttggccggaacatgtggggtgttgcttctctcccttgtgatcactctgtattgtaagcgcgggagaaagaagctcctgtacatcttcaagcagccttttatgcgacctgtgcaaaccactcaggaagaagatgggtgttcatgccgcttccccgaggaggaagaaggagggtgtgaactgagggtgaaattttctagaagcgccgatgctcccgcatatcagcagggtcagaatcagctctacaatgaattgaatctcggcaggcgagaagagtacgatgttctggacaagagacggggcagggatcccgagatggggggaaagccccggagaaaaaatcctcaggaggggttgtacaatgagctgcagaaggacaagatggctgaagcctatagcgagatcggaatgaaaggcgaaagacgcagaggcaaggggcatgacggtctgtaccagggtctctctacagccaccaaggacacttatgatgcgttgcatatgcaagccttgccaccccgctaagcggccgcgctttatttgtgaaatttgtgatgctattgctttatttgtaaccattataagctgcaataaacaagttaacaacaacaattgcattcattttatgtttcaggttcagggggagatgtgggaggttttttaaagctcaccggttctgggcggtgctacaactgggctggcggccaggatggttcttaggtaggtggggtcggcggtcaggtgtcccagagccaggggtctggagggaccttccaccctcagtccctggcaggtcggggggtgctgaggcgggcctggccctggcagcccaggggtcccggagcgaggggtctggagggacctttcactctcagtccctggcaggtcggggggtgctgtggcaggcccagccttggcccccagctctgccccttaccctgagctgtgtggctttgggcagctcgaactcctgggttcctctctgggccccaactcctcccctggcccaagtcccctctttgctcctgggcaggcaggacctctgtcccctctcagccggtccttggggctgcgtgtttctgtagaatgacgggtcaggctggccagaaccccaaaccttggccgtggggagtctgcgtggcggctctgccttgcccaggcatccttggtcctcactcgagttttcctaaggatgggatgagccccatgtgggactaaccttggctttacgacgtcaaagtttagatgagctggtgatatttttctcattatatccaaagtgtacctgttcgagtgaggacagttcttctgtctccaggatccctcctgggtggggattgtgcccgcctgggtctctgcccagattccagggctctccccgagccctgttcagaccatccgtgggggaggccttggcctcactcttacgtagataagtagcatggcgggttaatcattaactacaaggaacccctagtgatggagttggccactccctctctgcgcgctcgctcgctcactgaggccgggcgaccaaaggtcgcccgacgcccgggctttgcccgggcggcctcagtgagcgagcgagcgcgccagctggcgtaatagcgaagaggcccgcaccgatcgcccttcccaacagttgcgcagcctgaatggcgaatggcgattccgttgcaatggctggcggtaatattgttctggatattaccagcaaggccgatagtttgagttcttctactcaggcaagtgatgttattactaatcaaagaagtattgcgacaacggttaatttgcgtgatggacagactcttttactcggtggcctcactgattataaaaacacttctcaggattctggcgtaccgttcctgtctaaaatccctttaatcggcctcctgtttagctcccgctctgattctaacgaggaaagcacgttatacgtgctcgtcaaagcaaccatagtacgcgccctgtagcggcgcattaagcgcggcgggtgtggtggttacgcgcagcgtgaccgctacacttgccagcgccctagcgcccgctcctttcgctttcttcccttcctttctcgccacgttcgccggctttccccgtcaagctctaaatcgggggctccctttagggttccgatttagtgctttacggcacctcgaccccaaaaaacttgattagggtgatggttcacgtagtgggccatcgccctgatagacggtttttcgccctttgacgttggagtccacgttctttaatagtggactcttgttccaaactggaacaacactcaaccctatctcggtctattcttttgatttataagggattttgccgatttcggcctattggttaaaaaatgagctgatttaacaaaaatttaacgcgaattttaacaaaatattaacgtttacaatttaaatatttgcttatacaatcttcctgtttttggggcttttctgattatcaaccggggtacatatgattgacatgctagttttacgattaccgttcatcgattctcttgtttgctccagactctcaggcaatgacctgatagcctttgtagagacctctcaaaaatagctaccctctccggcatgaatttatcagctagaacggttgaatatcatattgatggtgatttgactgtctccggcctttctcacccgtttgaatctttacctacacattactcaggcattgcatttaaaatatatgagggttctaaaaatttttatccttgcgttgaaataaaggcttctcccgcaaaagtattacagggtcataatgtttttggtacaaccgatttagctttatgctctgaggctttattgcttaattttgctaattctttgccttgcctgtatgatttattggatgttggaatcgcctgatgcggtattttctccttacgcatctgtgcggtatttcacaccgcatatggtgcactctcagtacaatctgctctgatgccgcatagttaagccagccccgacacccgccaacacccgctgacgcgccctgacgggcttgtctgctcccggcatccgcttacagacaagctgtgaccgtctccgggagctgcatgtgtcagaggttttcaccgtcatcaccgaaacgcgcgagacgaaagggcctcgtgatacgcctatttttataggttaatgtcatgataataatggtttcttagacgtcaggtggcacttttcggggaaatgtgcgcggaacccctatttgtttatttttctaaatacattcaaatatgtatccgctcatgagacaataaccctgataaatgcttcaataatattgaaaaaggaagagtatgagtattcaacatttccgtgtcgcccttattcccttttttgcggcattttgccttcctgtttttgctcacccagaaacgctggtgaaagtaaaagatgctgaagatcagttgggtgcacgagtgggttacatcgaactggatctcaacagcggtaagatccttgagagttttcgccccgaagaacgttttccaatgatgagcacttttaaagttctgctatgtggcgcggtattatcccgtattgacgccgggcaagagcaactcggtcgccgcatacactattctcagaatgacttggttgagtactcaccagtcacagaaaagcatcttacggatggcatgacagtaagagaattatgcagtgctgccataaccatgagtgataacactgcggccaacttacttctgacaacgatcggaggaccgaaggagctaaccgcttttttgcacaacatgggggatcatgtaactcgccttgatcgttgggaaccggagctgaatgaagccataccaaacgacgagcgtgacaccacgatgcctgtagcaatggcaacaacgttgcgcaaactattaactggcgaactacttactctagcttcccggcaacaattaatagactggatggaggcggataaagttgcaggaccacttctgcgctcggcccttccggctggctggtttattgctgataaatctggagccggtgagcgtgggtctcgcggtatcattgcagcactggggccagatggtaagccctcccgtatcgtagttatctacacgacggggagtcaggcaactatggatgaacgaaatagacagatcgctgagataggtgcctcactgattaagcattggtaactgtcagaccaagtttactcatatatactttagattgatttaaaacttcatttttaatttaaaaggatctaggtgaagatcctttttgataatctcatgaccaaaatcccttaacgtgagttttcgttccactgagcgtcagaccccgtagaaaagatcaaaggatcttcttgagatcctttttttctgcgcgtaatctgctgcttgcaaacaaaaaaaccaccgctaccagcggtggtttgtttgccggatcaagagctaccaactctttttccgaaggtaactggcttcagcagagcgcagataccaaatactgtccttctagtgtagccgtagttaggccaccacttcaagaactctgtagcaccgcctacatacctcgctctgctaatcctgttaccagtggctgctgccagtggcgataagtcgtgtcttaccgggttggactcaagacgatagttaccggataaggcgcagcggtcgggctgaacggggggttcgtgcacacagcccagcttggagcgaacgacctacaccgaactgagatacctacagcgtgagctatgagaaagcgccacgcttcccgaagggagaaaggcggacaggtatccggtaagcggcagggtcggaacaggagagcgcacgagggagcttccagggggaaacgcctggtatctttatagtcctgtcgggtttcgccacctctgacttgagcgtcgatttttgtgatgctcgtcaggggggcggagcctatggaaaaacgccagcaacgcggcctttttacggttcctggccttttgctggccttttgctcacatgttctttcctgcgttatcccctgattctgtggataaccgtattaccgcctttgagtgagctgataccgctcgccgcagccgaacgaccgagcgcagcgagtcagtgagcgaggaagcggaagagcgcccaatacgcaaaccgcctctccccgcgcgttggccgattcattaatg

SEQ ID NO: 58 - DNA, 6147 bp, Artificial Sequence
  Synthesized rAAV PD-1 Exon1_ATG-mCherry construct
cagctgcgcgctcgctcgctcactgaggccgcccgggcaaagcccgggcgtcgggcgacctttggtcgcccggcctcagtgagcgagcgagcgcgcagagagggagtggccaactccatcactaggggttccttgtagttaatgattaacccgccatgctacttatctacgtaaggctgttgcaggcatcacacggtggaaagatctggaactgtggccatggtgtgaggccatccacaaggtggaagctttgagggggagccgattagccatggacagttgtcattcagtagggtcacctgtgccccagcgaagggggatgggccgggaaggcagaggccaggcacctgcccccagcaggggcagaggctgtgggcagccgggaggctcccagaggctccgacagaatgggagtggggttgagcccacccctcactgcagcccaggaacctgagcccagagggggccacccaccttccccaggcagggaggcccggcccccagggagatgggggggatgggggaggagaagggcctgcccccacccggcagcctcaggaggggcagctcgggcgggatatggaaagaggccacagcagtgagcagagacacagaggaggaaggggccctgagctggggagacccccacggggtagggcgtgggggccacgggcccacctcctccccatctcctctgtctccctgtctctgtctctctctccctcccccaccctctccccagtcctaccccctcctcacccctcctcccccagcactgcctctgtcactctcgcccacgtggatgtggaggaagagggggcgggagcaaggggcgggcaccctcccttcaacctgacctgggacagtttcccttccgctcacctccgcctgagcagtggagaaggcggcactctggtggggctgctccaggcatgcaggtgagcaagggcgaggaggataactccgccatcatcaaggagttcctgcgcttcaaggtgcacatggagggctccgtgaacggccacgagttcgagatcgagggcgagggcgagggccgcccctacgagggcacccagaccgccaagctgaaggtgaccaagggtggccccctgcccttcgcctgggacatcctgtcccctcagttcatgtacggctccaaggcctacgtgaagcaccccgccgacatccccgactacttgaagctgtccttccccgagggcttcaagtgggagcgcgtgatgaacttcgaggacggcggcgtggtgaccgtgacccaggactcctctctgcaggacggcgagttcatctacaaggtgaagctgcgcggcaccaacttcccctccgacggccccgtaatgcagaagaagaccatgggctgggaggcctcctccgagcggatgtaccccgaggacggcgccctgaagggcgagatcaagcagaggctgaagctgaaggacggcggccactacgacgctgaggtcaagaccacctacaaggccaagaagcccgtgcagctgcccggcgcctacaacgtcaacatcaagttggacatcacctcccacaacgaggactacaccatcgtggaacagtacgaacgcgccgagggccgccactccaccggcggcatggacgagctgtacaagtgatgaaagctttgctttatttgtgaaatttgtgatgctatgctttatttgtaaccattataagctgcaataaacaagtttaacaacaacaattgcattcattttatgtttcaggttcagggggaggtgtgggaggttttttaaagtaggtggggtcggcggtcaggtgtcccagagccaggggtctggagggaccttccaccctcagtccctggcaggtcggggggtgctgaggcgggcctggccctggcagcccaggggtcccggagcgaggggtctggagggacctttcactctcagtccctggcaggtcggggggtgctgtggcaggcccagccttggcccccagctctgccccttaccctgagctgtgtggctttgggcagctcgaactcctgggttcctctctgggccccaactcctcccctggcccaagtcccctctttgctcctgggcaggcaggacctctgtcccctctcagccggtccttggggctgcgtgtttctgtagaatgacgggtcaggctggccagaaccccaaaccttggccgtggggagtctgcgtggcggctctgccttgcccaggcatccttggtcctcactcgagttttcctaaggatgggatgagccccatgtgggactaaccttggctttacgacgtcaaagtttagatgagctggtgatatttttctcattatatccaaagtgtacctgttcgagtgaggacagttcttctgtctccaggatacgtagataagtagcatggcgggttaatcattaactacaaggaacccctagtgatggagttggccactccctctctgcgcgctcgctcgctcactgaggccgggcgaccaaaggtcgcccgacgcccgggctttgcccgggcggcctcagtgagcgagcgagcgcgccagctggcgtaatagcgaagaggcccgcaccgatcgcccttcccaacagttgcgcagcctgaatggcgaatggcgattccgttgcaatggctggcggtaatattgttctggatattaccagcaaggccgatagtttgagttcttctactcaggcaagtgatgttattactaatcaaagaagtattgcgacaacggttaatttgcgtgatggacagactcttttactcggtggcctcactgattataaaaacacttctcaggattctggcgtaccgttcctgtctaaaatccctttaatcggcctcctgtttagctcccgctctgattctaacgaggaaagcacgttatacgtgctcgtcaaagcaaccatagtacgcgccctgtagcggcgcattaagcgcggcgggtgtggtggttacgcgcagcgtgaccgctacacttgccagcgccctagcgcccgctcctttcgctttcttcccttcctttctcgccacgttcgccggctttccccgtcaagctctaaatcgggggctccctttagggttccgatttagtgctttacggcacctcgaccccaaaaaacttgattagggtgatggttcacgtagtgggccatcgccctgatagacggtttttcgccctttgacgttggagtccacgttctttaatagtggactcttgttccaaactggaacaacactcaaccctatctcggtctattcttttgatttataagggattttgccgatttcggcctattggttaaaaaatgagctgatttaacaaaaatttaacgcgaattttaacaaaatattaacgtttacaatttaaatatttgcttatacaatcttcctgtttttggggcttttctgattatcaaccggggtacatatgattgacatgctagttttacgattaccgttcatcgattctcttgtttgctccagactctcaggcaatgacctgatagcctttgtagagacctctcaaaaatagctaccctctccggcatgaatttatcagctagaacggttgaatatcatattgatggtgatttgactgtctccggcctttctcacccgtttgaatctttacctacacattactcaggcattgcatttaaaatatatgagggttctaaaaatttttatccttgcgttgaaataaaggcttctcccgcaaaagtattacagggtcataatgtttttggtacaaccgatttagctttatgctctgaggctttattgcttaattttgctaattctttgccttgcctgtatgatttattggatgttggaatcgcctgatgcggtattttctccttacgcatctgtgcggtatttcacaccgcatatggtgcactctcagtacaatctgctctgatgccgcatagttaagccagccccgacacccgccaacacccgctgacgcgccctgacgggcttgtctgctcccggcatccgcttacagacaagctgtgaccgtctccgggagctgcatgtgtcagaggttttcaccgtcatcaccgaaacgcgcgagacgaaagggcctcgtgatacgcctatttttataggttaatgtcatgataataatggtttcttagacgtcaggtggcacttttcggggaaatgtgcgcggaacccctatttgtttatttttctaaatacattcaaatatgtatccgctcatgagacaataaccctgataaatgcttcaataatattgaaaaaggaagagtatgagtattcaacatttccgtgtcgcccttattcccttttttgcggcattttgccttcctgtttttgctcacccagaaacgctggtgaaagtaaaagatgctgaagatcagttgggtgcacgagtgggttacatcgaactggatctcaacagcggtaagatccttgagagttttcgccccgaagaacgttttccaatgatgagcacttttaaagttctgctatgtggcgcggtattatcccgtattgacgccgggcaagagcaactcggtcgccgcatacactattctcagaatgacttggttgagtactcaccagtcacagaaaagcatcttacggatggcatgacagtaagagaattatgcagtgctgccataaccatgagtgataacactgcggccaacttacttctgacaacgatcggaggaccgaaggagctaaccgcttttttgcacaacatgggggatcatgtaactcgccttgatcgttgggaaccggagctgaatgaagccataccaaacgacgagcgtgacaccacgatgcctgtagcaatggcaacaacgttgcgcaaactattaactggcgaactacttactctagcttcccggcaacaattaatagactggatggaggcggataaagttgcaggaccacttctgcgctcggcccttccggctggctggtttattgctgataaatctggagccggtgagcgtgggtctcgcggtatcattgcagcactggggccagatggtaagccctcccgtatcgtagttatctacacgacggggagtcaggcaactatggatgaacgaaatagacagatcgctgagataggtgcctcactgattaagcattggtaactgtcagaccaagtttactcatatatactttagattgatttaaaacttcatttttaatttaaaaggatctaggtgaagatcctttttgataatctcatgaccaaaatcccttaacgtgagttttcgttccactgagcgtcagaccccgtagaaaagatcaaaggatcttcttgagatcctttttttctgcgcgtaatctgctgcttgcaaacaaaaaaaccaccgctaccagcggtggtttgtttgccggatcaagagctaccaactctttttccgaaggtaactggcttcagcagagcgcagataccaaatactgtccttctagtgtagccgtagttaggccaccacttcaagaactctgtagcaccgcctacatacctcgctctgctaatcctgttaccagtggctgctgccagtggcgataagtcgtgtcttaccgggttggactcaagacgatagttaccggataaggcgcagcggtcgggctgaacggggggttcgtgcacacagcccagcttggagcgaacgacctacaccgaactgagatacctacagcgtgagctatgagaaagcgccacgcttcccgaagggagaaaggcggacaggtatccggtaagcggcagggtcggaacaggagagcgcacgagggagcttccagggggaaacgcctggtatctttatagtcctgtcgggtttcgccacctctgacttgagcgtcgatttttgtgatgctcgtcaggggggcggagcctatggaaaaacgccagcaacgcggcctttttacggttcctggccttttgctggccttttgctcacatgttctttcctgcgttatcccctgattctgtggataaccgtattaccgcctttgagtgagctgataccgctcgccgcagccgaacgaccgagcgcagcgagtcagtgagcgaggaagcggaagagcgcccaatacgcaaaccgcctctccccgcgcgttggccgattcattaatg

SEQ ID NO: 59 - protein, 232 aa, Artificial Sequence
  Made in Lab
MQIPQAPWPVVWAVLQLGWRPGWFLDSPDRPWNPPTFSPALLVVTEGDNATFTCSFSNTSESFVLNWYRMSPSNQTDKLAAFPEDRSQPGQDCRFRVTQLPNGRDFHMSVVRARRNDSGTYLCGAISLAPKAQIKESLRAELRVTERRAEVPTAHPSPSPRPAGQFQTLVVGVVGGLLGSLVLLVWVLAVIRSKRSRLLHSDYMNMTPRRPGPTRKHYQPYAPPRDFAAYRS

SEQ ID NO: 60 - protein, 303 aa, Artificial Sequence; identical to SEQ ID NO: 6
  Synthesized I-OnuI variant PD-1.ile3.exon1_RD2_B1G2
  MOD_RES (1)..(4): Any amino acid or absent
  MOD_RES (302)..(303): Any amino acid or absent

SEQ ID NO: 61 - protein, 303 aa, Artificial Sequence
  Synthesized I-OnuI variant PD-1.ile3.exon1_RD3_B1G2C4
  MOD_RES (1)..(4): Any amino acid or absent
  MOD_RES (302)..(303): Any amino acid or absent
XXXXSRRESINPWILTGFADAEGSFGLSILNRNRGTARYHTRLSFTIMLHNKDKSILENIQSTWKVGSILNNGDHYVSLVVYRFEDLKVIIDHFEKYPLITQKLGDYKLFKQAFSVMENKEHLKENGIKELVRIKAKMNWGLNDELKKAFPENISKERPLINKNIPNFKWLAGFTSGDGSFFVRLRKSNVNARVRVQLVFEISQHIRDKNLMNSLITYLGCGHIYEGNKSERSWLQFRVEKFSDINDKIIPVFQENTLIGVKLEDFEDWCKVAKLIEEKKHLTESGLDEIKKIKLNMNKGRXX

SEQ ID NO: 62 - protein, 303 aa, Artificial Sequence
  Synthesized I-OnuI variant PD-1.ile3.exon1_RD3_B1 G2C11
  MOD_RES (1)..(4): Any amino acid or absent
  MOD_RES (302)..(303): Any amino acid or absent
XXXXSRRESINPWILTGFADAEGSFGLSILNRNRGTGRYHTRLSFTIMLHNKDKSILENIQSTWKVGSITNNGDHYVSLVVYRFEDLKVIIDHFEKYPLITQKLGDYKLFKQAFSVMENKEHLKENGIKELVRIKAKMNWGLNDELKKAFPENISKERPLINKNIPNFKWLAGFTSGDGSFFVRLRKSNVNARVRVQLVFEISQHIRDKNLMNSLITYLGCGHIYEGNKSERSWLQFRVEKFSDINDKIIPVFQENTLIGVKLEDFEDWCKVAKLIEEKKHLTESGLDEIKKIKLNMNKGRXX

SEQ ID NO: 63 - protein, 303 aa, Artificial Sequence
  Synthesized I-OnuI variant PD-1.ile3.exon1_RD3_B1 G2C5
  MOD_RES (1)..(4): Any amino acid or absent
  MOD_RES (302)..(303): Any amino acid or absent
XXXXSRRESINPWILTGFADAEGSFGLSILNRNRGTARYHTRLSFTIMLHNKDKSILENIQSTWKVGSIYNNGDHYVSLEVFRFEDLKVIIDHFEKYPLITQKLGDYKLFKQAFSVMENKEHLKENGIKELVRIKAKMNWGLNDELKKAFPENISKERPLINKNIPNFKWLAGFTSGDGSFFVRLRKSNVNARVRVQLVFEISQHIRDKNLMNSLITYLGCGHIYEGNKSERSWLQFRVEKFSDINDKIIPVFQENTLIGVKLEDFEDWCKVAKLIEEKKHLTESGLDEIKKIKLNMNKGRXX

SEQ ID NO: 64 - protein, 943 aa, Artificial Sequence
  Synthesized megaTAL PD-1.ile3.exon1_RD1_B1G2 construct
MGSAPPKKKRKVVDLRTLGYSQQQQEKIKPKVRSTVAQHHEALVGHGFTHAHIVALSQHPAALGTVAVTYQHIITALPEATHEDIVGVGKQWSGARALEALLTDAGELRGPPLQLDTGQLVKIAKRGGVTAMEAVHASRNALTGAPLNLTPDQVVAIASNNGGKQALETVQRLLPVLCQDHGLTPDQVVAIASNNGGKQALETVQRLLPVLCQDHGLTPDQVVAIASNGGGKQALETVQRLLPVLCQDHGLTPDQVVAIASNNGGKQALETVQRLLPVLCQDHGLTPDQVVAIASNNGGKQALETVQRLLPVLCQDHGLTPDQVVAIASNNGGKQALETVQRLLPVLCQDHGLTPDQVVAIASNNGGKQALETVQRLLPVLCQDHGLTPDQVVAIASHDGGKQALETVQRLLPVLCQDHGLTPDQVVAIASNGGGKQALETVQRLLPVLCQDHGLTPDQVVAIASNNGGKQALETVQRLLPVLCQDHGLTPDQVVAIASHDGGKQALETVQRLLPVLCQDHGLTPDQVVAIASNGGGKQALETVQRLLPVLCQDHGLTPDQVVAIASHDGGKQALESIVAQLSRPDPALAALTNDHLVALACLGGRPAMDAVKKGLPHAPELIRRVNRRIGERTSHRVAISRVGGSSRRESINPWILTGFADAEGSFGLSILNRNRGTARYHTRLSFTIMLHNKDKSILENIQSTWKVGIITNNGDHYVTLRVTRFEDLKVIIDHFEKYPLVTQKLGDYKLFKQAFSVMENKEHLKENGIKELVRIKAKMNWGLNDELKKAFPENISKERPLINKNIPNFKWLAGFTSGDGSFFVRLRKSNVNARVRVQLVFEISQHIRDKNLMNSLITYLGCGHIYEGNKSERSWLQFRVEKFSDINDKIIPVFQENTLIGVKLEDFEDWCKVAKLIEEKKHLTESGLDEIKKIKLNMNKGR

SEQ ID NO: 65 - RNA, 2832 nt, Artificial Sequence
  Synthesized PD-1 Exon1 RD2_B1G2 megaTAL mRNA construct
augggaagcgcgccaccuaagaagaaacgcaaagucguggaucuacgcacgcucggcuacagucagcagcagcaagagaagaucaaaccgaaggugcguucgacaguggcgcagcaccacgaggcacuggugggccauggguuuacacacgcgcacaucguugcgcucagccaacacccggcagcguuagggaccgucgcugucacguaucagcacauaaucacggcguugccagaggcgacacacgaagacaucguuggcgucggcaaacagugguccggcgcacgcgcccuggaggccuugcucacggaugcgggggaguugagagguccgccguuacaguuggacacaggccaacuugugaagauugcaaaacguggcggcgugaccgcaauggaggcagugcaugcaucgcgcaaugcacugacgggugccccccugaaccuaaccccugaucagguagucgcuauagcuucaaacaacgggggcaagcaagcacuggagaccguucaacgacuccugccagugcucugccaagaccacggacuuacgccagaucaggugguugcuauugccuccaacaauggcgggaaacaagcguuggaaacugugcagagacuguuaccugucuugugucaagaccacggccucacgccagaucaggugguagccauagcgucgaauggaggugguaagcaagcccuugaaacgguccagcgucuucugccgguguugugccaggaccacggacuaacgccggaucaggucguagccauugcuucaaauaacggcggcaaacaggcgcuagagacaguccagcgccucuugccuguguuaugccaggaucacggcuuaaccccagaccaaguuguggcuauugcaucuaacaaugguggcaaacaagccuuggagacagugcaacgauuacugccugucuuaugucaggaucauggccugacgcccgaucagguaguggcaaucgcaucuaauaauggagguaagcaagcacuggagacuguccagagauuguuacccguacuaugucaagaucaugguuugacgccugaucagguuguugcgauagccagcaacaacggagggaaacaggcucuugaaaccguacagcgacuucucccagucuugugccaagaucacgggcuuacuccugaucaagucguagcuaucgccagccacgacggugggaaacaggcccuggaaaccguacaacgucuccucccaguacuuugucaagaccacggguugacuccggaucaagucgucgcgaucgcgagcaauggaggggggaagcaggcgcuggaaacuguucagagacugcugccuguacuuugucaggaccauggucugacaccugaccaaguuguggcgauagccaguaacaaugggggaaaacaggcacuagagacgguucaaagguuguugcccguucugugccaggaccacggcuugacaccggaucaggugguagcuaucgcuucacacgauggcggaaaacaggcuuuagaaacaguccaaagacuucucccaguccuuugucaggaccacggauugacuccagaucaagucguugcuauugcaaguaaugguggugguaagcaagcuuuagaaaccguacagaggcuuuugccagugcugugccaggaccauggacugaccccugaucaagugguagcaauugcaucucaugauggaggaaaacaagcucuggaaagcauuguggcccagcugagccggccugauccggcguuggccgcguugaccaacgaccaccucgucgccuuggccugccucggcggacguccugccauggaugcagugaaaaagggauugccgcacgcgccggaauugaucagaagagucaaucgccguauuggcgaacgcacgucccaucgcguugcgauaucuagagugggaggaagcucucgcagagaguccaucaacccauggauucugacugguuucgcugaugccgaaggaucauucgggcuaagcauccucaacagaaacagagguacugcuagauaccacacucgacugucauucacaaucaugcugcacaacaaggacaaaucgauucuggagaauauccagucgacuuggaaggucggcauaaucaccaacaacggcgaccacuacgucacccugcgcgucacccguuucgaagauuugaaagugauuaucgaccacuucgagaaauauccgcugguaacacagaaauugggcgauuacaaguuguuuaaacaggcauucagcgucauggagaacaaagaacaucuuaaggagaaugggauuaaggagcucguacgaaucaaagcuaagaugaauuggggucucaaugacgaauugaaaaaagcauuuccagagaacauuagcaaagagcgcccccuuaucaauaagaacauuccgaauuucaaauggcuggcuggauucacaucuggugauggcuccuucuucgugcgccuaagaaagucuaauguuaaugcuagaguacgugugcaacugguauucgagaucucacagcacaucagagacaagaaccugaugaauucauugauaacauaccuaggcuguggucacaucuacgagggaaacaaaucugagcgcaguuggcuccaauucagaguagaaaaauucagcgauaucaacgacaagaucauuccgguauuccaggaaaauacucugauuggcgucaaacucgaggacuuugaagauuggugcaagguugccaaauugaucgaagagaagaaacaccugaccgaauccgguuuggaugagauuaagaaaaucaagcugaacaugaacaaaggucguuga

SEQ ID NO: 66 - RNA, 2832 nt, Artificial Sequence
  Synthesized PD-1 Exon1 RD2_B1G2C4 megaTAL mRNA construct
augggaagcgcgccaccuaagaagaaacgcaaagucguggaucuacgcacgcucggcuacagucagcagcagcaagagaagaucaaaccgaaggugcguucgacaguggcgcagcaccacgaggcacuggugggccauggguuuacacacgcgcacaucguugcgcucagccaacacccggcagcguuagggaccgucgcugucacguaucagcacauaaucacggcguugccagaggcgacacacgaagacaucguuggcgucggcaaacagugguccggcgcacgcgcccuggaggccuugcucacggaugcgggggaguugagagguccgccguuacaguuggacacaggccaacuugugaagauugcaaaacguggcggcgugaccgcaauggaggcagugcaugcaucgcgcaaugcacugacgggugccccccugaaccuaaccccugaucagguagucgcuauagcuucaaacaacgggggcaagcaagcacuggagaccguucaacgacuccugccagugcucugccaagaccacggacuuacgccagaucaggugguugcuauugccuccaacaauggcgggaaacaagcguuggaaacugugcagagacuguuaccugucuugugucaagaccacggccucacgccagaucaggugguagccauagcgucgaauggaggugguaagcaagcccuugaaacgguccagcgucuucugccgguguugugccaggaccacggacuaacgccggaucaggucguagccauugcuucaaauaacggcggcaaacaggcgcuagagacaguccagcgccucuugccuguguuaugccaggaucacggcuuaaccccagaccaaguuguggcuauugcaucuaacaaugguggcaaacaagccuuggagacagugcaacgauuacugccugucuuaugucaggaucauggccugacgcccgaucagguaguggcaaucgcaucuaauaauggagguaagcaagcacuggagacuguccagagauuguuacccguacuaugucaagaucaugguuugacgccugaucagguuguugcgauagccagcaacaacggagggaaacaggcucuugaaaccguacagcgacuucucccagucuugugccaagaucacgggcuuacuccugaucaagucguagcuaucgccagccacgacggugggaaacaggcccuggaaaccguacaacgucuccucccaguacuuugucaagaccacggguugacuccggaucaagucgucgcgaucgcgagcaauggaggggggaagcaggcgcuggaaacuguucagagacugcugccuguacuuugucaggaccauggucugacaccugaccaaguuguggcgauagccaguaacaaugggggaaaacaggcacuagagacgguucaaagguuguugcccguucugugccaggaccacggcuugacaccggaucaggugguagcuaucgcuucacacgauggcggaaaacaggcuuuagaaacaguccaaagacuucucccaguccuuugucaggaccacggauugacuccagaucaagucguugcuauugcaaguaaugguggugguaagcaagcuuuagaaaccguacagaggcuuuugccagugcugugccaggaccauggacugaccccugaucaagugguagcaauugcaucucaugauggaggaaaacaagcucuggaaagcauuguggcccagcugagccggccugauccggcguuggccgcguugaccaacgaccaccucgucgccuuggccugccucggcggacguccugccauggaugcagugaaaaagggauugccgcacgcgccggaauugaucagaagagucaaucgccguauuggcgaacgcacgucccaucgcguugcgauaucuagagugggaggaagcucucgcagagaguccaucaacccauggauucugacugguuucgcugaugccgaaggaucauucgggcuaagcauccucaacagaaacagagguacugcuagauaccacacucgacugucauucacaaucaugcugcacaacaaggacaaaucgauucuggagaauauccagucgacuuggaaggucggcagcauccucaacaauggcgaccacuacgucucgcugguggucuaccguuucgaagauuugaaagugauuaucgaccacuucgagaaauauccgcugauaacacagaaauugggcgauuacaaguuguuuaaacaggcauucagcgucauggagaacaaagaacaucuuaaggagaaugggauuaaggagcucguacgaaucaaagcuaagaugaauuggggucucaaugacgaauugaaaaaagcauuuccagagaacauuagcaaagagcgcccccuuaucaauaagaacauuccgaauuucaaauggcuggcuggauucacaucuggugauggcuccuucuucgugcgccuaagaaagucuaauguuaaugcuagaguacgugugcaacugguauucgagaucucacagcacaucagagacaagaaccugaugaauucauugauaacauaccuaggcuguggucacaucuacgagggaaacaaaucugagcgcaguuggcuccaauucagaguagaaaaauucagcgauaucaacgacaagaucauuccgguauuccaggaaaauacucugauuggcgucaaacucgaggacuuugaagauuggugcaagguugccaaauugaucgaagagaagaaacaccugaccgaauccgguuuggaugagauuaagaaaaucaagcugaacaugaacaaaggucguuga

SEQ ID NO: 67 - RNA, 2832 nt, Artificial Sequence
  Synthesized PD-1 Exon1 RD2_B1G2C11 megaTAL mRNA construct
augggaagcgcgccaccuaagaagaaacgcaaagucguggaucuacgcacgcucggcuacagucagcagcagcaagagaagaucaaaccgaaggugcguucgacaguggcgcagcaccacgaggcacuggugggccauggguuuacacacgcgcacaucguugcgcucagccaacacccggcagcguuagggaccgucgcugucacguaucagcacauaaucacggcguugccagaggcgacacacgaagacaucguuggcgucggcaaacagugguccggcgcacgcgcccuggaggccuugcucacggaugcgggggaguugagagguccgccguuacaguuggacacaggccaacuugugaagauugcaaaacguggcggcgugaccgcaauggaggcagugcaugcaucgcgcaaugcacugacgggugccccccugaaccuaaccccugaucagguagucgcuauagcuucaaacaacgggggcaagcaagcacuggagaccguucaacgacuccugccagugcucugccaagaccacggacuuacgccagaucaggugguugcuauugccuccaacaauggcgggaaacaagcguuggaaacugugcagagacuguuaccugucuugugucaagaccacggccucacgccagaucaggugguagccauagcgucgaauggaggugguaagcaagcccuugaaacgguccagcgucuucugccgguguugugccaggaccacggacuaacgccggaucaggucguagccauugcuucaaauaacggcggcaaacaggcgcuagagacaguccagcgccucuugccuguguuaugccaggaucacggcuuaaccccagaccaaguuguggcuauugcaucuaacaaugguggcaaacaagccuuggagacagugcaacgauuacugccugucuuaugucaggaucauggccugacgcccgaucagguaguggcaaucgcaucuaauaauggagguaagcaagcacuggagacuguccagagauuguuacccguacuaugucaagaucaugguuugacgccugaucagguuguugcgauagccagcaacaacggagggaaacaggcucuugaaaccguacagcgacuucucccagucuugugccaagaucacgggcuuacuccugaucaagucguagcuaucgccagccacgacggugggaaacaggcccuggaaaccguacaacgucuccucccaguacuuugucaagaccacggguugacuccggaucaagucgucgcgaucgcgagcaauggaggggggaagcaggcgcuggaaacuguucagagacugcugccuguacuuugucaggaccauggucugacaccugaccaaguuguggcgauagccaguaacaaugggggaaaacaggcacuagagacgguucaaagguuguugcccguucugugccaggaccacggcuugacaccggaucaggugguagcuaucgcuucacacgauggcggaaaacaggcuuuagaaacaguccaaagacuucucccaguccuuugucaggaccacggauugacuccagaucaagucguugcuauugcaaguaaugguggugguaagcaagcuuuagaaaccguacagaggcuuuugccagugcugugccaggaccauggacugaccccugaucaagugguagcaauugcaucucaugauggaggaaaacaagcucuggaaagcauuguggcccagcugagccggccugauccggcguuggccgcguugaccaacgaccaccucgucgccuuggccugccucggcggacguccugccauggaugcagugaaaaagggauugccgcacgcgccggaauugaucagaagagucaaucgccguauuggcgaacgcacgucccaucgcguugcgauaucuagagugggaggaagcucucgcagagaguccaucaacccauggauucugacugguuucgcugaugccgaaggaucauucgggcuaagcauccucaacagaaacagagguacugguagauaccacacucgacugucauucacaaucaugcugcacaacaaggacaaaucgauucuggagaauauccagucgacuuggaaggucggcucgaucacgaacaacggcgaccacuacgucagccuggucgucuaccguuucgaagauuugaaagugauuaucgaccacuucgagaaauauccgcugauaacacagaaauugggcgauuacaaguuguuuaaacaggcauucagcgucauggagaacaaagaacaucuuaaggagaaugggauuaaggagcucguacgaaucaaagcuaagaugaauuggggucucaaugacgaauugaaaaaagcauuuccagagaacauuagcaaagagcgcccccuuaucaauaagaacauuccgaauuucaaauggcuggcuggauucacaucuggugauggcuccuucuucgugcgccuaagaaagucuaauguuaaugcuagaguacgugugcaacugguauucgagaucucacagcacaucagagacaagaaccugaugaauucauugauaacauaccuaggcuguggucacaucuacgagggaaacaaaucugagcgcaguuggcuccaauucagaguagaaaaauucagcgauaucaacgacaagaucauuccgguauuccaggaaaauacucugauuggcgucaaacucgaggacuuugaagauuggugcaagguugccaaauugaucgaagagaagaaacaccugaccgaauccgguuuggaugagauuaagaaaaucaagcugaacaugaacaaaggucguuga

SEQ ID NO: 68 - RNA, 2832 nt, Artificial Sequence
  Synthesized PD-1 Exon1 RD2_B1G2C5 megaTAL mRNA construct
augggaagcgcgccaccuaagaagaaacgcaaagucguggaucuacgcacgcucggcuacagucagcagcagcaagagaagaucaaaccgaaggugcguucgacaguggcgcagcaccacgaggcacuggugggccauggguuuacacacgcgcacaucguugcgcucagccaacacccggcagcguuagggaccgucgcugucacguaucagcacauaaucacggcguugccagaggcgacacacgaagacaucguuggcgucggcaaacagugguccggcgcacgcgcccuggaggccuugcucacggaugcgggggaguugagagguccgccguuacaguuggacacaggccaacuugugaagauugcaaaacguggcggcgugaccgcaauggaggcagugcaugcaucgcgcaaugcacugacgggugccccccugaaccuaaccccugaucagguagucgcuauagcuucaaacaacgggggcaagcaagcacuggagaccguucaacgacuccugccagugcucugccaagaccacggacuuacgccagaucaggugguugcuauugccuccaacaauggcgggaaacaagcguuggaaacugugcagagacuguuaccugucuugugucaagaccacggccucacgccagaucaggugguagccauagcgucgaauggaggugguaagcaagcccuugaaacgguccagcgucuucugccgguguugugccaggaccacggacuaacgccggaucaggucguagccauugcuucaaauaacggcggcaaacaggcgcuagagacaguccagcgccucuugccuguguuaugccaggaucacggcuuaaccccagaccaaguuguggcuauugcaucuaacaaugguggcaaacaagccuuggagacagugcaacgauuacugccugucuuaugucaggaucauggccugacgcccgaucagguaguggcaaucgcaucuaauaauggagguaagcaagcacuggagacuguccagagauuguuacccguacuaugucaagaucaugguuugacgccugaucagguuguugcgauagccagcaacaacggagggaaacaggcucuugaaaccguacagcgacuucucccagucuugugccaagaucacgggcuuacuccugaucaagucguagcuaucgccagccacgacggugggaaacaggcccuggaaaccguacaacgucuccucccaguacuuugucaagaccacggguugacuccggaucaagucgucgcgaucgcgagcaauggaggggggaagcaggcgcuggaaacuguucagagacugcugccuguacuuugucaggaccauggucugacaccugaccaaguuguggcgauagccaguaacaaugggggaaaacaggcacuagagacgguucaaagguuguugcccguucugugccaggaccacggcuugacaccggaucaggugguagcuaucgcuucacacgauggcggaaaacaggcuuuagaaacaguccaaagacuucucccaguccuuugucaggaccacggauugacuccagaucaagucguugcuauugcaaguaaugguggugguaagcaagcuuuagaaaccguacagaggcuuuugccagugcugugccaggaccauggacugaccccugaucaagugguagcaauugcaucucaugauggaggaaaacaagcucuggaaagcauuguggcccagcugagccggccugauccggcguuggccgcguugaccaacgaccaccucgucgccuuggccugccucggcggacguccugccauggaugcagugaaaaagggauugccgcacgcgccggaauugaucagaagagucaaucgccguauuggcgaacgcacgucccaucgcguugcgauaucuagagugggaggaagcucucgcagagaguccaucaacccauggauucugacugguuucgcugaugccgaaggaucauucgggcuaagcauccucaacagaaacagagguacugcuagauaccacacucgacugucauucacaaucaugcugcacaacaaggacaaaucgauucuggagaauauccagucgacuuggaaggucggcucgaucuacaacaacggcgaccacuacgucucgcuggaggucuuccguuucgaagauuugaaagugauuaucgaccacuucgagaaauauccgcugauaacacagaaauugggcgauuacaaguuguuuaaacaggcauucagcgucauggagaacaaagaacaucuuaaggagaaugggauuaaggagcucguacgaaucaaagcuaagaugaauuggggucucaaugacgaauugaaaaaagcauuuccagagaacauuagcaaagagcgcccccuuaucaauaagaacauuccgaauuucaaauggcuggcuggauucacaucuggugauggcuccuucuucgugcgccuaagaaagucuaauguuaaugcuagaguacgugugcaacugguauucgagaucucacagcacaucagagacaagaaccugaugaauucauugauaacauaccuaggcuguggucacaucuacgagggaaacaaaucugagcgcaguuggcuccaauucagaguagaaaaauucagcgauaucaacgacaagaucauuccgguauuccaggaaaauacucugauuggcgucaaacucgaggacuuugaagauuggugcaagguugccaaauugaucgaagagaagaaacaccugaccgaauccgguuuggaugagauuaagaaaaucaagcugaacaugaacaaaggucguuga

SEQ ID NO: 69 - protein, 3 aa, Artificial Sequence
  Exemplary linker sequence
GGG

SEQ ID NO: 70 - protein, 5 aa, Artificial Sequence
  Exemplary linker sequence
DGGGS

SEQ ID NO: 71 - protein, 5 aa, Artificial Sequence
  Exemplary linker sequence
TGEKP

SEQ ID NO: 72 - protein, 4 aa, Artificial Sequence
  Exemplary linker sequence
GGRR

SEQ ID NO: 73 - protein, 5 aa, Artificial Sequence
  Exemplary linker sequence
GGGGS

SEQ ID NO: 74 - protein, 14 aa, Artificial Sequence
  Exemplary linker sequence
EGKSSGSGSESKVD

SEQ ID NO: 75 - protein, 18 aa, Artificial Sequence
  Exemplary linker sequence
KESGSVSSEQLAQFRSLD

SEQ ID NO: 76 - protein, 8 aa, Artificial Sequence
  Exemplary linker sequence
GGRRGGGS

SEQ ID NO: 77 - protein, 9 aa, Artificial Sequence
  Exemplary linker sequence
LRQRDGERP

SEQ ID NO: 78 - protein, 12 aa, Artificial Sequence
  Exemplary linker sequence
LRQKDGGGSERP

SEQ ID NO: 79 - protein, 16 aa, Artificial Sequence
  Exemplary linker sequence
LRQKDGGGSGGGSERP

SEQ ID NO: 80 - protein, 7 aa, Artificial Sequence
  Cleavage sequence by TEV protease
  misc_feature (2)..(3): Xaa is any amino acid
  misc_feature (5)..(5): Xaa is any amino acid
  MISC_FEATURE (7)..(7): Xaa = Gly or Ser
EXXYXQX

SEQ ID NO: 81 - protein, 7 aa, Artificial Sequence
  Cleavage sequence by TEV protease
ENLYFQG

SEQ ID NO: 82 - protein, 7 aa, Artificial Sequence
  Cleavage sequence by TEV protease
ENLYFQS

SEQ ID NO: 83 - protein, 22 aa, Artificial Sequence
  Self-cleaving polypeptide comprising 2A site
GSGATNFSLLKQAGDVEENPGP

SEQ ID NO: 84 - protein, 19 aa, Artificial Sequence
  Self-cleaving polypeptide comprising 2A site
ATNFSLLKQAGDVEENPGP

SEQ ID NO: 85 - protein, 14 aa, Artificial Sequence
  Self-cleaving polypeptide comprising 2A site
LLKQAGDVEENPGP

SEQ ID NO: 86 - protein, 21 aa, Artificial Sequence
  Self-cleaving polypeptide comprising 2A site
GSGEGRGSLLTCGDVEENPGP

SEQ ID NO: 87 - protein, 18 aa, Artificial Sequence
  Self-cleaving polypeptide comprising 2A site
EGRGSLLTCGDVEENPGP

SEQ ID NO: 88 - protein, 13 aa, Artificial Sequence
  Self-cleaving polypeptide comprising 2A site
LLTCGDVEENPGP

SEQ ID NO: 89 - protein, 23 aa, Artificial Sequence
  Self-cleaving polypeptide comprising 2A site
GSGQCTNYALLKLAGDVESNPGP

SEQ ID NO: 90 - protein, 20 aa, Artificial Sequence
  Self-cleaving polypeptide comprising 2A site
QCTNYALLKLAGDVESNPGP

SEQ ID NO: 91 - protein, 14 aa, Artificial Sequence
  Self-cleaving polypeptide comprising 2A site
LLKLAGDVESNPGP

SEQ ID NO: 92 - protein, 25 aa, Artificial Sequence
  Self-cleaving polypeptide comprising 2A site
GSGVKQTLNFDLLKLAGDVESNPGP

SEQ ID NO: 93 - protein, 22 aa, Artificial Sequence
  Self-cleaving polypeptide comprising 2A site
VKQTLNFDLLKLAGDVESNPGP

SEQ ID NO: 94 - protein, 14 aa, Artificial Sequence
  Self-cleaving polypeptide comprising 2A site
LLKLAGDVESNPGP

SEQ ID NO: 95 - protein, 19 aa, Artificial Sequence
  Self-cleaving polypeptide comprising 2A site
LLNFDLLKLAGDVESNPGP

SEQ ID NO: 96 - protein, 19 aa, Artificial Sequence
  Self-cleaving polypeptide comprising 2A site
TLNFDLLKLAGDVESNPGP

SEQ ID NO: 97 - protein, 14 aa, Artificial Sequence
  Self-cleaving polypeptide comprising 2A site
LLKLAGDVESNPGP

SEQ ID NO: 98 - protein, 17 aa, Artificial Sequence
  Self-cleaving polypeptide comprising 2A site
NFDLLKLAGDVESNPGP

SEQ ID NO: 99 - protein, 20 aa, Artificial Sequence
  Self-cleaving polypeptide comprising 2A site
QLLNFDLLKLAGDVESNPGP

SEQ ID NO: 100 - protein, 24 aa, Artificial Sequence
  Self-cleaving polypeptide comprising 2A site
APVKQTLNFDLLKLAGDVESNPGP

SEQ ID NO: 101 - protein, 40 aa, Artificial Sequence
  Self-cleaving polypeptide comprising 2A site
VTELLYRMKRAETYCPRPLLAIHPTEARHKQKIVAPVKQT

SEQ ID NO: 102 - protein, 18 aa, Artificial Sequence
  Self-cleaving polypeptide comprising 2A site
LNFDLLKLAGDVESNPGP

SEQ ID NO: 103 - protein, 40 aa, Artificial Sequence
  Self-cleaving polypeptide comprising 2A site
LLAIHPTEARHKQKIVAPVKQTLNFDLLKLAGDVESNPGP

SEQ ID NO: 104 - protein, 33 aa, Artificial Sequence
  Self-cleaving polypeptide comprising 2A site
EARHKQKIVAPVKQTLNFDLLKLAGDVESNPGP

SEQ ID NO: 105 - DNA, 10 bp, Artificial Sequence
  Consensus Kozak sequence
gccrccatgg

SEQ ID NO: 106 - protein, 8 aa, Homo sapiens
EQTEYATI

SEQ ID NO: 107 - DNA, 43 bp, Homo sapiens
tgagcagacggagtatgccaccattgtctttcctagcggaatg

SEQ ID NO: 108 - DNA, 43 bp, Artificial Sequence
  Made in Lab
cattccgctaggaaagacaatggtggcatactccgtctgctca

SEQ ID NO: 109 - DNA, 22 bp, Artificial Sequence
  Made in Lab
  misc_feature (14)..(22): n is A, C, G or T
aatggtggcatacnnnnnnnnn

SEQ ID NO: 110 - DNA, 22 bp, Artificial Sequence
  Made in Lab
  misc_feature (1)..(9): n is a, c, g, or t
nnnnnnnnnatactccgtctgc

SEQ ID NO: 111 - DNA, 22 bp, Artificial Sequence
  Made in Lab
aatggtggcatactccgtctgc

SEQ ID NO: 112 - DNA, 43 bp, Homo sapiens
attccgctaggaaagacaatggtggcatactccgtctgctcag

SEQ ID NO: 113 - DNA, 43 bp, Artificial Sequence
  Made in Lab
atttcgttaggaaagataatggtggtatatttcgtttgtttag

SEQ ID NO: 114 - protein, 7 aa, Homo sapiens
MQIPQAP

SEQ ID NO: 115 - DNA, 44 bp, Homo sapiens
ctctggtggggctgctccaggcatgcagatcccacaggcgccct

SEQ ID NO: 116 - DNA, 44 bp, Artificial Sequence
  Made in Lab
agggcgcctgtgggatctgcatccctggagcagccccaccagag

SEQ ID NO: 117 - protein, 8 aa, Homo sapiens
NGRDFHMS

SEQ ID NO: 118 - DNA, 43 bp, Homo sapiens
gtgtcacacaactgcccaacgggcgtgacttccacatgagcgt

SEQ ID NO: 119 - DNA, 43 bp, Artificial Sequence
  Made in Lab
acgctcatgtggaagtcacgcccgttgggcagttgtgtgacac

SEQ ID NO: 120 - DNA, 32 bp, Homo sapiens
gctccaggcatgcagatcccacaggcgccctg

SEQ ID NO: 121 - DNA, 32 bp, Artificial Sequence
  made in lab
actccaaacatacaaatcccacaaacacccta

SEQ ID NO: 122 - DNA, 31 bp, Homo sapiens
gcccaacgggcgtgacttccacatgagcgtg

SEQ ID NO: 123 - DNA, 31 bp, Artificial Sequence
  Made in Lab
acccaacgaacgtaacttccacataaacgta